European Patent Specification EP 4 189 087 B1, published November 15, 2023. Title: RNA molecule, use thereof and a process for detecting a disease by using thereof. Applicant: Moirai Biodesign, S.L. The sequence listing filed with the application follows.

SEQUENCE LISTING (86 sequences)

SEQ ID NO: 1 - RNA, 30 nt, artificial
  Artificial
guccaacagcgccagagaacaacuaugaug

SEQ ID NO: 2 - RNA, 30 nt, artificial
  Artificial
cgccgcuggcccggguuggauaauauuuag

SEQ ID NO: 3 - DNA, 2799 bp, escherichia coli
atgcacggttacgatgcgcccatctacaccaacgtgacctatcccattacggtcaatccgccgtttgttcccacggagaatccgacgggttgttactcgctcacatttaatgttgatgaaagctggctacaggaaggccagacgcgaattatttttgatggcgttaactcggcgtttcatctgtggtgcaacgggcgctgggtcggttacggccaggacagtcgtttgccgtctgaatttgacctgagcgcatttttacgcgccggagaaaaccgcctcgcggtgatggtgctgcgctggagtgacggcagttatctggaagatcaggatatgtggcggatgagcggcattttccgtgacgtctcgttgctgcataaaccgactacacaaatcagcgatttccatgttgccactcgctttaatgatgatttcagccgcgctgtactggaggctgaagttcagatgtgcggcgagttgcgtgactacctacgggtaacagtttctttatggcagggtgaaacgcaggtcgccagcggcaccgcgcctttcggcggtgaaattatcgatgagcgtggtggttatgccgatcgcgtcacactacgtctgaacgtcgaaaacccgaaactgtggagcgccgaaatcccgaatctctatcgtgcggtggttgaactgcacaccgccgacggcacgctgattgaagcagaagcctgcgatgtcggtttccgcgaggtgcggattgaaaatggtctgctgctgctgaacggcaagccgttgctgattcgaggcgttaaccgtcacgagcatcatcctctgcatggtcaggtcatggatgagcagacgatggtgcaggatatcctgctgatgaagcagaacaactttaacgccgtgcgctgttcgcattatccgaaccatccgctgtggtacacgctgtgcgaccgctacggcctgtatgtggtggatgaagccaatattgaaacccacggcatggtgccaatgaatcgtctgaccgatgatccgcgctggctaccggcgatgagcgaacgcgtaacgcgaatggtgcagcgcgatcgtaatcacccgagtgtgatcatctggtcgctggggaatgaatcaggccacggcgctaatcacgacgcgctgtatcgctggatcaaatctgtcgatccttcccgcccggtgcagtatgaaggcggcggagccgacaccacggccaccgatattatttgcccgatgtacgcgcgcgtggatgaagaccagcccttcccggctgtgccgaaatggtccatcaaaaaatggctttcgctacctggagagacgcgcccgctgatcctttgcgaatacgcccacgcgatgggtaacagtcttggcggtttcgctaaatactggcaggcgtttcgtcagtatccccgtttacagggcggcttcgtctgggactgggtggatcagtcgctgattaaatatgatgaaaacggcaacccgtggtcggcttacggcggtgattttggcgatacgccgaacgatcgccagttctgtatgaacggtctggtctttgccgaccgcacgccgcatccagcgctgacggaagcaaaacaccagcagcagtttttccagttccgtttatccgggcaaaccatcgaagtgaccagcgaatacctgttccgtcatagcgataacgagctcctgcactggatggtggcgctggatggtaagccgctggcaagcggtgaagtgcctctggatgtcgctccacaaggtaaacagttgattgaactgcctgaactaccgcagccggagagcgccgggcaactctggctcacagtacgcgtagtgcaaccgaacgcgaccgcatggtcagaagccgggcacatcagcgcctggcagcagtggcgtctggcggaaaacctcagtgtgacgctccccgccgcgtcccacgccatcccgcatctgaccaccagcgaaatggatttttgcatcgagctgggtaataagcgttggcaatttaaccgccagtcaggctttctttcacagatgtggattggcgataaaaaacaactgctgacgccgctgcgcgatcagttcacccgtgcaccgctggataacgacattggcgtaagtgaagcgacccgcattgaccctaacgcctgggtcgaacgctggaaggcggcgggccattaccaggccgaagcagcgttgttgcagtgcacggcagatacacttgctgatgcggtgctgattacgaccgctcacgcgtggcagcatcaggggaaaaccttatttatcagccggaaaacctaccggattgatggtagtggtcaaatggcgattaccgttgatgttgaagtggcgagcgatacaccgcatccggcgcggattggcctgaactgccagctggcgcaggtagcagagcgggtaaactggctcggattagggccgcaagaaaactatcccgaccgccttactgccgcctgttttgaccgctgggatctgccattgtcagacatgtataccccgtacgtcttcccgagcgaaaacggtctgcgctgcgggacgcgcgaattgaattatggcccacaccagtggcgcggcgacttccagttcaacatcagccgctacagtcaacagcaactgatggaaaccagccatcgccatctgctgcacgcggaagaaggcacatggctgaatatcgacggtttccatatggggattggtggcgacgactcctggagcccgtcagtatcggcggaattccagctgagcgccggtcgctaccattaccagttggtctggtgtcaaaaataa

SEQ ID NO: 4 - RNA, 160 nt, artificial
  Artificial
ggccaucauaguuguucucuggcgcuguuggacgaaaacaguccagcagcgccgggaaggaggggcgaggcauaaguuccuccuucuuggcguuguuggaccuaagaaggaggaauuuaugucauaucucacacaacgggaggucguuuuacaacgucgu

SEQ ID NO: 5 - RNA, 160 nt, artificial
  Artificial
ggccaucauaguuguucucuggcgcuguuggacgaaaacaguccagcagcgccgggaaggaggggcgagagauaaguuccuccuucuuggcguuguuggaccuaagaaggaggaauuuaugucauaucucacacaacgggaggucguuuuacaacgucgu

SEQ ID NO: 6 - RNA, 160 nt, Artificial Sequence
  Artificial
ggccuaaauauuauccaacccgggccagcggcggauaaaaugucguugguccgggagagggaggcgugaaaaaauugucuuucuuuuucggauuaaugauacgaaaaaggaggauaucauguacuacagcuucgaucccgccgucguuuuacaacgucgu

SEQ ID NO: 7 - DNA, 7964 bp, Artificial Sequence
  Artificial
gaattcgagctcggtacccggggatcctctagagtcgacctgcaggcatgcaagcttcgatcccgccgtcgttttacaacgtcgtgactgggaaaaccctggcgttacccaacttaatcgccttgcagcacatccccctttcgccagctggcgtaatagcgaagaggcccgcaccgatcgcccttcccaacagttgcgcagcctgaatggcgaatggcgctttgcctggtttccggcaccagaagcggtgccggaaagctggctggagtgcgatcttcctgaggccgatactgtcgtcgtcccctcaaactggcagatgcacggttacgatgcgcccatctacaccaacgtaacctatcccattacggtcaatccgccgtttgttcccacggagaatccgacgggttgttactcgctcacatttaatgttgatgaaagctggctacaggaaggccagacgcgaattatttttgatggcgttaactcggcgtttcatctgtggtgcaacgggcgctgggtcggttacggccaggacagtcgtttgccgtctgaatttgacctgagcgcatttttacgcgccggagaaaaccgcctcgcggtgatggtgctgcgttggagtgacggcagttatctggaagatcaggatatgtggcggatgagcggcattttccgtgacgtctcgttgctgcataaaccgactacacaaatcagcgatttccatgttgccactcgctttaatgatgatttcagccgcgctgtactggaggctgaagttcagatgtgcggcgagttgcgtgactacctacgggtaacagtttctttatggcagggtgaaacgcaggtcgccagcggcaccgcgcctttcggcggtgaaattatcgatgagcgtggtggttatgccgatcgcgtcacactacgtctgaacgtcgaaaacccgaaactgtggagcgccgaaatcccgaatctctatcgtgcggtggttgaactgcacaccgccgacggcacgctgattgaagcagaagcctgcgatgtcggtttccgcgaggtgcggattgaaaatggtctgctgctgctgaacggcaagccgttgctgattcgaggcgttaaccgtcacgagcatcatcctctgcatggtcaggtcatggatgagcagacgatggtgcaggatatcctgctgatgaagcagaacaactttaacgccgtgcgctgttcgcattatccgaaccatccgctgtggtacacgctgtgcgaccgctacggcctgtatgtggtggatgaagccaatattgaaacccacggcatggtgccaatgaatcgtctgaccgatgatccgcgctggctaccggcgatgagcgaacgcgtaacgcgaatggtgcagcgcgatcgtaatcacccgagtgtgatcatctggtcgctggggaatgaatcaggccacggcgctaatcacgacgcgctgtatcgctggatcaaatctgtcgatccttcccgcccggtgcagtatgaaggcggcggagccgacaccacggccaccgatattatttgcccgatgtacgcgcgcgtggatgaagaccagcccttcccggctgtgccgaaatggtccatcaaaaaatggctttcgctacctggagagacgcgcccgctgatcctttgcgaatacgcccacgcgatgggtaacagtcttggcggtttcgctaaatactggcaggcgtttcgtcagtatccccgtttacagggcggcttcgtctgggactgggtggatcagtcgctgattaaatatgatgaaaacggcaacccgtggtcggcttacggcggtgattttggcgatacgccgaacgatcgccagttctgtatgaacggtctggtctttgccgaccgcacgccgcatccagcgctgacggaagcaaaacaccagcagcagtttttccagttccgtttatccgggcaaaccatcgaagtgaccagcgaatacctgttccgtcatagcgataacgagctcctgcactggatggtggcgctggatggtaagccgctggcaagcggtgaagtgcctctggatgtcgctccacaaggtaaacagttgattgaactgcctgaactaccgcagccggagagcgccgggcaactctggctcacagtacgcgtagtgcaaccgaacgcgaccgcatggtcagaagccgggcacatcagcgcctggcagcagtggcgtctggcggaaaacctcagtgtgacgctccccgccgcgtcccacgccatcccgcatctgaccaccagcgaaatggatttttgcatcgagctgggtaataagcgttggcaatttaaccgccagtcaggctttctttcacagatgtggattggcgataaaaaacaactgctgacgccgctgcgcgatcagttcacccgtgcaccgctggataacgacattggcgtaagtgaagcgacccgcattgaccctaacgcctgggtcgaacgctggaaggcggcgggccattaccaggccgaagcagcgttgttgcagtgcacggcagatacacttgctgatgcggtgctgattacgaccgctcacgcgtggcagcatcaggggaaaaccttatttatcagccggaaaacctaccggattgatggtagtggtcaaatggcgattaccgttgatgttgaagtggcgagcgatacaccgcatccggcgcggattggcctgaactgccagctggcgcaggtagcagagcgggtaaactggctcggattagggccgcaagaaaactatcccgaccgccttactgccgcctgttttgaccgctgggatctgccattgtcagacatgtataccccgtacgtcttcccgagcgaaaacggtctgcgctgcgggacgcgcgaattgaattatggcccacaccagtggcgcggcgacttccagttcaacatcagccgctacagtcaacagcaactgatggaaaccagccatcgccatctgctgcacgcggaagaaggcacatggctgaatatcgacggtttccatatggggattggtggcgacgactcctggagcccgtcagtatcggcggaattacagctgagcgccggtcgctaccattaccagttggtctggtgtcaaaaataataataaccgggcaggccatgtctgcccgtatttcgcgtaaggaaatccattatgtactatttcgcctgatgcggtattttctccttacgcatctgtgcggtatttcacaccgcatagggtaataactgatataattaaattgaagctctaatttgtgagtttagtatacatgcatttacttataatacagttttttagttttgctggccgcatcttctcaaatatgcttcccagcctgcttttctgtaacgttcaccctctaccttagcatcccttccctttgcaaatagtcctcttccaacaataataatgtcagatcctgtagagaccacatcatccacggttctatactgttgacccaatgcgtctcccttgtcatctaaacccacaccgggtgtcataatcaaccaatcgtaaccttcatctcttccacccatgtctctttgagcaataaagccgataacaaaatctttgtcgctcttcgcaatgtcaacagtacccttagtatattctccagtagatagggagcccttgcatgacaattctgctaacatcaaaaggcctctaggttcctttgttacttcttctgccgcctgcttcaaaccgctaacaatacctgggcccaccacaccgtgtgcattcgtaatgtctgcccattctgctattctgtatacacccgcagagtactgcaatttgactgtattaccaatgtcagcaaattttctgtcttcgaagagtaaaaaattgtacttggcggataatgcctttagcggcttaactgtgccctccatggaaaaatcagtcaagatatccacatgtgtttttagtaaacaaattttgggacctaatgcttcaactaactccagtaattccttggtggtacgaacatccaatgaagcacacaagtttgtttgcttttcgtgcatgatattaaatagcttggcagcaacaggactaggatgagtagcagcacgttccttatatgtagctttcgacatgatttatcttcgttttttgttctgtgcagttgggttaagaatactgggcaatttcatgtttcttcaacactacatatgcgtatatataccaatctaagtctgtgctccttccttcgttcttccttctgttcggagattaccgaatcaaaaaaatttcaaagaaaccgaaatcaaaaaaaagaataaaaaaaaaatgatgaattgaattgaaaagctacttgttacccatcattgaattttgaacatccgaacctgggagttttccctgaaacagatagtatatttgaacctgtataataatatatagtctagcgctttacggaagacaatgtatgtatttcggttcctggagaaactattgcatctattgcataggtaatcttgcacgtcgcatccccggttcattttctgcgtttccatcttgcacttcaatagcatatctttgttaacgaagcatctgtgcttcattttgtagaacaaaaatgcaacgcgagagcgctaatttttcaaacaaagaatctgagctgcatttttacagaacagaaatgcaacgcgaaagcgctattttaccaacgaagaatctgtgcttcatttttgtaaaacaaaaatgcaacgcgagagcgctaatttttcaaacaaagaatctgagctgcatttttacagaacagaaatgcaacgcgagagcgctattttaccaacaaagaatctatacttcttttttgttctacaaaaatgcatcccgagagcgctatttttctaacaaagcatcttagattactttttttctcctttgtgcgctctataatgcagtctcttgataactttttgcactgtaggtccgttaaggttagaagaaggctactttggtgtctattttctcttccataaaaaaagcctgactccacttcccgcgtttactgattactagcgaagctgcgggtgcattttttcaagataaaggcatccccgattatattctataccgatgtggattgcgcatactttgtgaacagaaagtgatagcgttgatgattcttcattggtcagaaaattatgaacggtttcttctattttgtctctatatactacgtataggaaatgtttacattttcgtattgttttcgattcactctatgaatagttcttactacaatttttttgtctaaagagtaatactagagataaacataaaaaatgtagaggtcgagtttagatgcaagttcaaggagcgaaaggtggatgggtaggttatatagggatatagcacagagatatatagcaaagagatacttttgagcaatgtttgtggaagcggtattcgcaatattttagtagctcgttacagtccggtgcgtttttggttttttgaaagtgcgtcttcagagcgcttttggttttcaaaagcgctctgaagttcctatactttctagctagagaataggaacttcggaataggaacttcaaagcgtttccgaaaacgagcgcttccgaaaatgcaacgcgagctgcgcacatacagctcactgttcacgtcgcacctatatctgcgtgttgcctgtatatatatatacatgagaagaacggcatagtgcgtgtttatgcttaaatgcgttatggtgcactctcagtacaatctgctctgatgccgcatagttaagccagccccgacacccgccaacacccgctgacgcgccctgacgggcttgtctgctcccggcatccgcttacagacaagctgtgaccgtctccgggagctgcatgtgtcagaggttttcaccgtcatcaccgaaacgcgcgagacgaaagggcctcgtgatacgcctatttttataggttaatgtcatgataataatggtttcttagacgtcaggtggcacttttcggggaaatgtgcgcggaacccctatttgtttatttttctaaatacattcaaatatgtatccgctcatgagacaataaccctgataaatgcttcaataatattgaaaaaggaagagtatgagtattcaacatttccgtgtcgcccttattcccttttttgcggcattttgccttcctgtttttgctcacccagaaacgctggtgaaagtaaaagatgctgaagatcagttgggtgcacgagtgggttacatcgaactggatctcaacagcggtaagatccttgagagttttcgccccgaagaacgttttccaatgatgagcacttttaaagttctgctatgtggcgcggtattatcccgtattgacgccgggcaagagcaactcggtcgccgcatacactattctcagaatgacttggttgagtactcaccagtcacagaaaagcatcttacggatggcatgacagtaagagaattatgcagtgctgccataaccatgagtgataacactgcggccaacttacttctgacaacgatcggaggaccgaaggagctaaccgcttttttgcacaacatgggggatcatgtaactcgccttgatcgttgggaaccggagctgaatgaagccataccaaacgacgagcgtgacaccacgatgcctgtagcaatggcaacaacgttgcgcaaactattaactggcgaactacttactctagcttcccggcaacaattaatagactggatggaggcggataaagttgcaggaccacttctgcgctcggcccttccggctggctggtttattgctgataaatctggagccggtgagcgtgggtctcgcggtatcattgcagcactggggccagatggtaagccctcccgtatcgtagttatctacacgacggggagtcaggcaactatggatgaacgaaatagacagatcgctgagataggtgcctcactgattaagcattggtaactgtcagaccaagtttactcatatatactttagattgatttaaaacttcatttttaatttaaaaggatctaggtgaagatcctttttgataatctcatgaccaaaatcccttaacgtgagttttcgttccactgagcgtcagaccccgtagaaaagatcaaaggatcttcttgagatcctttttttctgcgcgtaatctgctgcttgcaaacaaaaaaaccaccgctaccagcggtggtttgtttgccggatcaagagctaccaactctttttccgaaggtaactggcttcagcagagcgcagataccaaatactgtccttctagtgtagccgtagttaggccaccacttcaagaactctgtagcaccgcctacatacctcgctctgctaatcctgttaccagtggctgctgccagtggcgataagtcgtgtcttaccgggttggactcaagacgatagttaccggataaggcgcagcggtcgggctgaacggggggttcgtgcacacagcccagcttggagcgaacgacctacaccgaactgagatacctacagcgtgagcattgagaaagcgccacgcttcccgaagggagaaaggcggacaggtatccggtaagcggcagggtcggaacaggagagcgcacgagggagcttccagggggaaacgcctggtatctttatagtcctgtcgggtttcgccacctctgacttgagcgtcgatttttgtgatgctcgtcaggggggcggagcctatggaaaaacgccagcaacgcggcctttttacggttcctggccttttgctggccttttgctcacatgttctttcctgcgttatcccctgattctgtggataaccgtattaccgcctttgagtgagctgataccgctcgccgcagccgaacgaccgagcgcagcgagtcagtgagcgaggaagcggaagagcgcccaatacgcaaaccgcctctccccgcgcgttggccgattcattcccg

SEQ ID NO: 8 - DNA, 56 bp, artificial
  Artificial
aaacccctccgtttagagaggggttatgctagttatttttgacaccagaccaactg

SEQ ID NO: 9 - DNA, 187 bp, artificial
  Artificial
tcataagctttaatacgactcactataggccatcatagttgttctctggcgctgttggacgaaaacagtccagcagcgccgggaaggaggggcgaggcataagttcctccttcttggcgttgttggacctaagaaggaggaatttatgtcatatctcacacaacgggaggtcgttttacaacgtcgt

SEQ ID NO: 10 - DNA, 187 bp, artificial
  Artificial
tcataagctttaatacgactcactataggccatcatagttgttctctggcgctgttggacgaaaacagtccagcagcgccgggaaggaggggcgagagataagttcctccttcttggcgttgttggacctaagaaggaggaatttatgtcatatctcacacaacgggaggtcgttttacaacgtcgt

SEQ ID NO: 11 - DNA, 187 bp, artificial
  Artificial
tcataagctttaatacgactcactataggcctaaatattatccaacccgggccagcggcggataaaatgtcgttggtccgggagagggaggcgtgaaaaaattgtctttctttttcggattaatgatacgaaaaaggaggatatcatgtactacagcttcgatcccgccgtcgttttacaacgtcgt

SEQ ID NO: 12 - DNA, 3249 bp, artificial
  Artificial
tcataagctttaatacgactcactataggccatcatagttgttctctggcgctgttggacgaaaacagtccagcagcgccgggaaggaggggcgaggcataagttcctccttcttggcgttgttggacctaagaaggaggaatttatgtcatatctcacacaacgggaggtcgttttacaacgtcgtgactgggaaaaccctggcgttacccaacttaatcgccttgcagcacatccccctttcgccagctggcgtaatagcgaagaggcccgcaccgatcgcccttcccaacagttgcgcagcctgaatggcgaatggcgctttgcctggtttccggcaccagaagcggtgccggaaagctggctggagtgcgatcttcctgaggccgatactgtcgtcgtcccctcaaactggcagatgcacggttacgatgcgcccatctacaccaacgtgacctatcccattacggtcaatccgccgtttgttcccacggagaatccgacgggttgttactcgctcacatttaatgttgatgaaagctggctacaggaaggccagacgcgaattatttttgatggcgttaactcggcgtttcatctgtggtgcaacgggcgctgggtcggttacggccaggacagtcgtttgccgtctgaatttgacctgagcgcatttttacgcgccggagaaaaccgcctcgcggtgatggtgctgcgctggagtgacggcagttatctggaagatcaggatatgtggcggatgagcggcattttccgtgacgtctcgttgctgcataaaccgactacacaaatcagcgatttccatgttgccactcgctttaatgatgatttcagccgcgctgtactggaggctgaagttcagatgtgcggcgagttgcgtgactacctacgggtaacagtttctttatggcagggtgaaacgcaggtcgccagcggcaccgcgcctttcggcggtgaaattatcgatgagcgtggtggttatgccgatcgcgtcacactacgtctgaacgtcgaaaacccgaaactgtggagcgccgaaatcccgaatctctatcgtgcggtggttgaactgcacaccgccgacggcacgctgattgaagcagaagcctgcgatgtcggtttccgcgaggtgcggattgaaaatggtctgctgctgctgaacggcaagccgttgctgattcgaggcgttaaccgtcacgagcatcatcctctgcatggtcaggtcatggatgagcagacgatggtgcaggatatcctgctgatgaagcagaacaactttaacgccgtgcgctgttcgcattatccgaaccatccgctgtggtacacgctgtgcgaccgctacggcctgtatgtggtggatgaagccaatattgaaacccacggcatggtgccaatgaatcgtctgaccgatgatccgcgctggctaccggcgatgagcgaacgcgtaacgcgaatggtgcagcgcgatcgtaatcacccgagtgtgatcatctggtcgctggggaatgaatcaggccacggcgctaatcacgacgcgctgtatcgctggatcaaatctgtcgatccttcccgcccggtgcagtatgaaggcggcggagccgacaccacggccaccgatattatttgcccgatgtacgcgcgcgtggatgaagaccagcccttcccggctgtgccgaaatggtccatcaaaaaatggctttcgctacctggagagacgcgcccgctgatcctttgcgaatacgcccacgcgatgggtaacagtcttggcggtttcgctaaatactggcaggcgtttcgtcagtatccccgtttacagggcggcttcgtctgggactgggtggatcagtcgctgattaaatatgatgaaaacggcaacccgtggtcggcttacggcggtgattttggcgatacgccgaacgatcgccagttctgtatgaacggtctggtctttgccgaccgcacgccgcatccagcgctgacggaagcaaaacaccagcagcagtttttccagttccgtttatccgggcaaaccatcgaagtgaccagcgaatacctgttccgtcatagcgataacgagctcctgcactggatggtggcgctggatggtaagccgctggcaagcggtgaagtgcctctggatgtcgctccacaaggtaaacagttgattgaactgcctgaactaccgcagccggagagcgccgggcaactctggctcacagtacgcgtagtgcaaccgaacgcgaccgcatggtcagaagccgggcacatcagcgcctggcagcagtggcgtctggcggaaaacctcagtgtgacgctccccgccgcgtcccacgccatcccgcatctgaccaccagcgaaatggatttttgcatcgagctgggtaataagcgttggcaatttaaccgccagtcaggctttctttcacagatgtggattggcgataaaaaacaactgctgacgccgctgcgcgatcagttcacccgtgcaccgctggataacgacattggcgtaagtgaagcgacccgcattgaccctaacgcctgggtcgaacgctggaaggcggcgggccattaccaggccgaagcagcgttgttgcagtgcacggcagatacacttgctgatgcggtgctgattacgaccgctcacgcgtggcagcatcaggggaaaaccttatttatcagccggaaaacctaccggattgatggtagtggtcaaatggcgattaccgttgatgttgaagtggcgagcgatacaccgcatccggcgcggattggcctgaactgccagctggcgcaggtagcagagcgggtaaactggctcggattagggccgcaagaaaactatcccgaccgccttactgccgcctgttttgaccgctgggatctgccattgtcagacatgtataccccgtacgtcttcccgagcgaaaacggtctgcgctgcgggacgcgcgaattgaattatggcccacaccagtggcgcggcgacttccagttcaacatcagccgctacagtcaacagcaactgatggaaaccagccatcgccatctgctgcacgcggaagaaggcacatggctgaatatcgacggtttccatatggggattggtggcgacgactcctggagcccgtcagtatcggcggaattccagctgagcgccggtcgctaccattaccagttggtctggtgtcaaaaataactagcataacccctctctaaacggaggggttt

SEQ ID NO: 13 - DNA, 3249 bp, artificial
  Artificial
tcataagctttaatacgactcactataggccatcatagttgttctctggcgctgttggacgaaaacagtccagcagcgccgggaaggaggggcgagagataagttcctccttcttggcgttgttggacctaagaaggaggaatttatgtcatatctcacacaacgggaggtcgttttacaacgtcgtgactgggaaaaccctggcgttacccaacttaatcgccttgcagcacatccccctttcgccagctggcgtaatagcgaagaggcccgcaccgatcgcccttcccaacagttgcgcagcctgaatggcgaatggcgctttgcctggtttccggcaccagaagcggtgccggaaagctggctggagtgcgatcttcctgaggccgatactgtcgtcgtcccctcaaactggcagatgcacggttacgatgcgcccatctacaccaacgtgacctatcccattacggtcaatccgccgtttgttcccacggagaatccgacgggttgttactcgctcacatttaatgttgatgaaagctggctacaggaaggccagacgcgaattatttttgatggcgttaactcggcgtttcatctgtggtgcaacgggcgctgggtcggttacggccaggacagtcgtttgccgtctgaatttgacctgagcgcatttttacgcgccggagaaaaccgcctcgcggtgatggtgctgcgctggagtgacggcagttatctggaagatcaggatatgtggcggatgagcggcattttccgtgacgtctcgttgctgcataaaccgactacacaaatcagcgatttccatgttgccactcgctttaatgatgatttcagccgcgctgtactggaggctgaagttcagatgtgcggcgagttgcgtgactacctacgggtaacagtttctttatggcagggtgaaacgcaggtcgccagcggcaccgcgcctttcggcggtgaaattatcgatgagcgtggtggttatgccgatcgcgtcacactacgtctgaacgtcgaaaacccgaaactgtggagcgccgaaatcccgaatctctatcgtgcggtggttgaactgcacaccgccgacggcacgctgattgaagcagaagcctgcgatgtcggtttccgcgaggtgcggattgaaaatggtctgctgctgctgaacggcaagccgttgctgattcgaggcgttaaccgtcacgagcatcatcctctgcatggtcaggtcatggatgagcagacgatggtgcaggatatcctgctgatgaagcagaacaactttaacgccgtgcgctgttcgcattatccgaaccatccgctgtggtacacgctgtgcgaccgctacggcctgtatgtggtggatgaagccaatattgaaacccacggcatggtgccaatgaatcgtctgaccgatgatccgcgctggctaccggcgatgagcgaacgcgtaacgcgaatggtgcagcgcgatcgtaatcacccgagtgtgatcatctggtcgctggggaatgaatcaggccacggcgctaatcacgacgcgctgtatcgctggatcaaatctgtcgatccttcccgcccggtgcagtatgaaggcggcggagccgacaccacggccaccgatattatttgcccgatgtacgcgcgcgtggatgaagaccagcccttcccggctgtgccgaaatggtccatcaaaaaatggctttcgctacctggagagacgcgcccgctgatcctttgcgaatacgcccacgcgatgggtaacagtcttggcggtttcgctaaatactggcaggcgtttcgtcagtatccccgtttacagggcggcttcgtctgggactgggtggatcagtcgctgattaaatatgatgaaaacggcaacccgtggtcggcttacggcggtgattttggcgatacgccgaacgatcgccagttctgtatgaacggtctggtctttgccgaccgcacgccgcatccagcgctgacggaagcaaaacaccagcagcagtttttccagttccgtttatccgggcaaaccatcgaagtgaccagcgaatacctgttccgtcatagcgataacgagctcctgcactggatggtggcgctggatggtaagccgctggcaagcggtgaagtgcctctggatgtcgctccacaaggtaaacagttgattgaactgcctgaactaccgcagccggagagcgccgggcaactctggctcacagtacgcgtagtgcaaccgaacgcgaccgcatggtcagaagccgggcacatcagcgcctggcagcagtggcgtctggcggaaaacctcagtgtgacgctccccgccgcgtcccacgccatcccgcatctgaccaccagcgaaatggatttttgcatcgagctgggtaataagcgttggcaatttaaccgccagtcaggctttctttcacagatgtggattggcgataaaaaacaactgctgacgccgctgcgcgatcagttcacccgtgcaccgctggataacgacattggcgtaagtgaagcgacccgcattgaccctaacgcctgggtcgaacgctggaaggcggcgggccattaccaggccgaagcagcgttgttgcagtgcacggcagatacacttgctgatgcggtgctgattacgaccgctcacgcgtggcagcatcaggggaaaaccttatttatcagccggaaaacctaccggattgatggtagtggtcaaatggcgattaccgttgatgttgaagtggcgagcgatacaccgcatccggcgcggattggcctgaactgccagctggcgcaggtagcagagcgggtaaactggctcggattagggccgcaagaaaactatcccgaccgccttactgccgcctgttttgaccgctgggatctgccattgtcagacatgtataccccgtacgtcttcccgagcgaaaacggtctgcgctgcgggacgcgcgaattgaattatggcccacaccagtggcgcggcgacttccagttcaacatcagccgctacagtcaacagcaactgatggaaaccagccatcgccatctgctgcacgcggaagaaggcacatggctgaatatcgacggtttccatatggggattggtggcgacgactcctggagcccgtcagtatcggcggaattccagctgagcgccggtcgctaccattaccagttggtctggtgtcaaaaataactagcataacccctctctaaacggaggggttt

SEQ ID NO: 14 - DNA, 3249 bp, artificial
  Artificial
tcataagctttaatacgactcactataggcctaaatattatccaacccgggccagcggcggataaaatgtcgttggtccgggagagggaggcgtgaaaaaattgtctttctttttcggattaatgatacgaaaaaggaggatatcatgtactacagcttcgatcccgccgtcgttttacaacgtcgtgactgggaaaaccctggcgttacccaacttaatcgccttgcagcacatccccctttcgccagctggcgtaatagcgaagaggcccgcaccgatcgcccttcccaacagttgcgcagcctgaatggcgaatggcgctttgcctggtttccggcaccagaagcggtgccggaaagctggctggagtgcgatcttcctgaggccgatactgtcgtcgtcccctcaaactggcagatgcacggttacgatgcgcccatctacaccaacgtgacctatcccattacggtcaatccgccgtttgttcccacggagaatccgacgggttgttactcgctcacatttaatgttgatgaaagctggctacaggaaggccagacgcgaattatttttgatggcgttaactcggcgtttcatctgtggtgcaacgggcgctgggtcggttacggccaggacagtcgtttgccgtctgaatttgacctgagcgcatttttacgcgccggagaaaaccgcctcgcggtgatggtgctgcgctggagtgacggcagttatctggaagatcaggatatgtggcggatgagcggcattttccgtgacgtctcgttgctgcataaaccgactacacaaatcagcgatttccatgttgccactcgctttaatgatgatttcagccgcgctgtactggaggctgaagttcagatgtgcggcgagttgcgtgactacctacgggtaacagtttctttatggcagggtgaaacgcaggtcgccagcggcaccgcgcctttcggcggtgaaattatcgatgagcgtggtggttatgccgatcgcgtcacactacgtctgaacgtcgaaaacccgaaactgtggagcgccgaaatcccgaatctctatcgtgcggtggttgaactgcacaccgccgacggcacgctgattgaagcagaagcctgcgatgtcggtttccgcgaggtgcggattgaaaatggtctgctgctgctgaacggcaagccgttgctgattcgaggcgttaaccgtcacgagcatcatcctctgcatggtcaggtcatggatgagcagacgatggtgcaggatatcctgctgatgaagcagaacaactttaacgccgtgcgctgttcgcattatccgaaccatccgctgtggtacacgctgtgcgaccgctacggcctgtatgtggtggatgaagccaatattgaaacccacggcatggtgccaatgaatcgtctgaccgatgatccgcgctggctaccggcgatgagcgaacgcgtaacgcgaatggtgcagcgcgatcgtaatcacccgagtgtgatcatctggtcgctggggaatgaatcaggccacggcgctaatcacgacgcgctgtatcgctggatcaaatctgtcgatccttcccgcccggtgcagtatgaaggcggcggagccgacaccacggccaccgatattatttgcccgatgtacgcgcgcgtggatgaagaccagcccttcccggctgtgccgaaatggtccatcaaaaaatggctttcgctacctggagagacgcgcccgctgatcctttgcgaatacgcccacgcgatgggtaacagtcttggcggtttcgctaaatactggcaggcgtttcgtcagtatccccgtttacagggcggcttcgtctgggactgggtggatcagtcgctgattaaatatgatgaaaacggcaacccgtggtcggcttacggcggtgattttggcgatacgccgaacgatcgccagttctgtatgaacggtctggtctttgccgaccgcacgccgcatccagcgctgacggaagcaaaacaccagcagcagtttttccagttccgtttatccgggcaaaccatcgaagtgaccagcgaatacctgttccgtcatagcgataacgagctcctgcactggatggtggcgctggatggtaagccgctggcaagcggtgaagtgcctctggatgtcgctccacaaggtaaacagttgattgaactgcctgaactaccgcagccggagagcgccgggcaactctggctcacagtacgcgtagtgcaaccgaacgcgaccgcatggtcagaagccgggcacatcagcgcctggcagcagtggcgtctggcggaaaacctcagtgtgacgctccccgccgcgtcccacgccatcccgcatctgaccaccagcgaaatggatttttgcatcgagctgggtaataagcgttggcaatttaaccgccagtcaggctttctttcacagatgtggattggcgataaaaaacaactgctgacgccgctgcgcgatcagttcacccgtgcaccgctggataacgacattggcgtaagtgaagcgacccgcattgaccctaacgcctgggtcgaacgctggaaggcggcgggccattaccaggccgaagcagcgttgttgcagtgcacggcagatacacttgctgatgcggtgctgattacgaccgctcacgcgtggcagcatcaggggaaaaccttatttatcagccggaaaacctaccggattgatggtagtggtcaaatggcgattaccgttgatgttgaagtggcgagcgatacaccgcatccggcgcggattggcctgaactgccagctggcgcaggtagcagagcgggtaaactggctcggattagggccgcaagaaaactatcccgaccgccttactgccgcctgttttgaccgctgggatctgccattgtcagacatgtataccccgtacgtcttcccgagcgaaaacggtctgcgctgcgggacgcgcgaattgaattatggcccacaccagtggcgcggcgacttccagttcaacatcagccgctacagtcaacagcaactgatggaaaccagccatcgccatctgctgcacgcggaagaaggcacatggctgaatatcgacggtttccatatggggattggtggcgacgactcctggagcccgtcagtatcggcggaattccagctgagcgccggtcgctaccattaccagttggtctggtgtcaaaaataactagcataacccctctctaaacggaggggttt

SEQ ID NO: 15 - DNA, 1450 bp, escherichia coli
agtttgatcatggctcagattgaacgctggcggcaggcctaacacatgcaagtcgaacggtaacaggaagcagcttgctgctttgctgacgagtggcggacgggtgagtaatgtctgggaaactgcctgatggagggggataactactggaaacggtagctaataccgcataacgtcgcaagcacaaagagggggaccttagggcctcttgccatcggatgtgcccagatgggattagctagtaggtggggtaacggctcacctaggcgacgatccctagctggtctgagaggatgaccagcaacactggaactgagacacggtccagactcctacgggaggcagcagtggggaatattgcacaatgggcgcaagcctgatgcagccatgccgcgtgtatgaagaaggccttcgggttgtaaagtactttcagcggggaggaagggagtaaagttaatacctttgctcattgacgttacccgcagaagaagcaccggctaactccgtgccagcagccgcggtaatacggagggtgcaagcgttaatcggaattactgggcgtaaagcgcacgcaggcggtttgttaagtcagatgtgaaatccccgggctcaacctgggaactgcatctgatactggcaagcttgagtctcgtagaggggggtagaattccaggtgtagcggtgaaatgcgtagagatctggaggaataccggtggcgaaggcggccccctggacgaagactgacgctcaggtgcgaaagcgtggggagcaaacaggattagataccctggtagtccacgccgtaaacgatgtcgacttggaggttgtgcccttgaggcgtggcttccggagctaacgcgttaagtcgaccgcctggggagtacggccgcaaggttaaaactcaaatgaattgacgggggccgcacaagcggtggagcatgtggtttaattcgatgcaacgcgaagaaccttacctggtcttgacatccacggaagttttcagagatgagaatgtgccttcgggaaccgtgagacaggtgctgcatggctgtcgtcagctcgtgttgtgaaatgttgggttaagtcccgcaacgagcgcaacccttatcctttgttgccagcggtccggccgggaactcaaaggagactgccagtgataaactggaggaaggtggggatgacgtcaagtcatcatggcccttacgaccagggctacacacgtgctacaatggcgcatacaaagagaagcgacctcgcgagagcaagcggacctcataaagtgcgtcgtagtccggattggagtctgcaactcgactccatgaagtcggaatcgctagtaatcgtggatcagaatgccacggtgaatacgttcccgggccttgtacacaccgcccgtcacaccatgggagtgggttgcaaaagaagtaggtagcttaacttcgggagggcg

SEQ ID NO: 16 - RNA, 159 nt, artificial
  Artificial
ggcguguaguugugcugcgugugugaggagggcugaaagagcucuuuucguauauaaaggaggguaccuauaaucuguccuccuuuauauacgaaaagaguauauaaaggaggacaauaugcacauacaaagcuucgaucccgccgucguuuuacaacg

SEQ ID NO: 17 - RNA, 159 nt, artificial
  Artificial
ggcguguaguugugcugcgugugugaggagggcugagagagcucuuuucguauauaaaggaggguaccuauaaucuguccuccuuuauauacgaaaagaguauauaaaggaggacaauaugcacauacaaagcuucgaucccgccgucguuuuacaacg

SEQ ID NO: 18 - RNA, 78 nt, escherichia coli
ugaaaguacuuuacaacccgaaggccuucuucauacacgcggcauggcugcaucaggcuuguugcgcccauucugcaa

SEQ ID NO: 19 - DNA, 186 bp, artificial
  Artificial
tcataagctttaatacgactcactataggcgtgtagttgtgctgcgtgtgtgaggagggctgaaagagctcttttcgtatataaaggagggtacctataatctgtcctcctttatatacgaaaagagtatataaaggaggacaatatgcacatacaaagcttcgatcccgccgtcgttttacaacg

SEQ ID NO: 20 - DNA, 186 bp, artificial
  Artificial
tcataagctttaatacgactcactataggcgtgtagttgtgctgcgtgtgtgaggagggctgagagagctcttttcgtatataaaggagggtacctataatctgtcctcctttatatacgaaaagagtatataaaggaggacaatatgcacatacaaagcttcgatcccgccgtcgttttacaacg

SEQ ID NO: 21 - DNA, 3252 bp, artificial
  Artificial
tcataagctttaatacgactcactataggcgtgtagttgtgctgcgtgtgtgaggagggctgaaagagctcttttcgtatataaaggagggtacctataatctgtcctcctttatatacgaaaagagtatataaaggaggacaatatgcacatacaaagcttcgatcccgccgtcgttttacaacgtcgtgactgggaaaaccctggcgttacccaacttaatcgccttgcagcacatccccctttcgccagctggcgtaatagcgaagaggcccgcaccgatcgcccttcccaacagttgcgcagcctgaatggcgaatggcgctttgcctggtttccggcaccagaagcggtgccggaaagctggctggagtgcgatcttcctgaggccgatactgtcgtcgtcccctcaaactggcagatgcacggttacgatgcgcccatctacaccaacgtgacctatcccattacggtcaatccgccgtttgttcccacggagaatccgacgggttgttactcgctcacatttaatgttgatgaaagctggctacaggaaggccagacgcgaattatttttgatggcgttaactcggcgtttcatctgtggtgcaacgggcgctgggtcggttacggccaggacagtcgtttgccgtctgaatttgacctgagcgcatttttacgcgccggagaaaaccgcctcgcggtgatggtgctgcgctggagtgacggcagttatctggaagatcaggatatgtggcggatgagcggcattttccgtgacgtctcgttgctgcataaaccgactacacaaatcagcgatttccatgttgccactcgctttaatgatgatttcagccgcgctgtactggaggctgaagttcagatgtgcggcgagttgcgtgactacctacgggtaacagtttctttatggcagggtgaaacgcaggtcgccagcggcaccgcgcctttcggcggtgaaattatcgatgagcgtggtggttatgccgatcgcgtcacactacgtctgaacgtcgaaaacccgaaactgtggagcgccgaaatcccgaatctctatcgtgcggtggttgaactgcacaccgccgacggcacgctgattgaagcagaagcctgcgatgtcggtttccgcgaggtgcggattgaaaatggtctgctgctgctgaacggcaagccgttgctgattcgaggcgttaaccgtcacgagcatcatcctctgcatggtcaggtcatggatgagcagacgatggtgcaggatatcctgctgatgaagcagaacaactttaacgccgtgcgctgttcgcattatccgaaccatccgctgtggtacacgctgtgcgaccgctacggcctgtatgtggtggatgaagccaatattgaaacccacggcatggtgccaatgaatcgtctgaccgatgatccgcgctggctaccggcgatgagcgaacgcgtaacgcgaatggtgcagcgcgatcgtaatcacccgagtgtgatcatctggtcgctggggaatgaatcaggccacggcgctaatcacgacgcgctgtatcgctggatcaaatctgtcgatccttcccgcccggtgcagtatgaaggcggcggagccgacaccacggccaccgatattatttgcccgatgtacgcgcgcgtggatgaagaccagcccttcccggctgtgccgaaatggtccatcaaaaaatggctttcgctacctggagagacgcgcccgctgatcctttgcgaatacgcccacgcgatgggtaacagtcttggcggtttcgctaaatactggcaggcgtttcgtcagtatccccgtttacagggcggcttcgtctgggactgggtggatcagtcgctgattaaatatgatgaaaacggcaacccgtggtcggcttacggcggtgattttggcgatacgccgaacgatcgccagttctgtatgaacggtctggtctttgccgaccgcacgccgcatccagcgctgacggaagcaaaacaccagcagcagtttttccagttccgtttatccgggcaaaccatcgaagtgaccagcgaatacctgttccgtcatagcgataacgagctcctgcactggatggtggcgctggatggtaagccgctggcaagcggtgaagtgcctctggatgtcgctccacaaggtaaacagttgattgaactgcctgaactaccgcagccggagagcgccgggcaactctggctcacagtacgcgtagtgcaaccgaacgcgaccgcatggtcagaagccgggcacatcagcgcctggcagcagtggcgtctggcggaaaacctcagtgtgacgctccccgccgcgtcccacgccatcccgcatctgaccaccagcgaaatggatttttgcatcgagctgggtaataagcgttggcaatttaaccgccagtcaggctttctttcacagatgtggattggcgataaaaaacaactgctgacgccgctgcgcgatcagttcacccgtgcaccgctggataacgacattggcgtaagtgaagcgacccgcattgaccctaacgcctgggtcgaacgctggaaggcggcgggccattaccaggccgaagcagcgttgttgcagtgcacggcagatacacttgctgatgcggtgctgattacgaccgctcacgcgtggcagcatcaggggaaaaccttatttatcagccggaaaacctaccggattgatggtagtggtcaaatggcgattaccgttgatgttgaagtggcgagcgatacaccgcatccggcgcggattggcctgaactgccagctggcgcaggtagcagagcgggtaaactggctcggattagggccgcaagaaaactatcccgaccgccttactgccgcctgttttgaccgctgggatctgccattgtcagacatgtataccccgtacgtcttcccgagcgaaaacggtctgcgctgcgggacgcgcgaattgaattatggcccacaccagtggcgcggcgacttccagttcaacatcagccgctacagtcaacagcaactgatggaaaccagccatcgccatctgctgcacgcggaagaaggcacatggctgaatatcgacggtttccatatggggattggtggcgacgactcctggagcccgtcagtatcggcggaattccagctgagcgccggtcgctaccattaccagttggtctggtgtcaaaaataactagcataacccctctctaaacggaggggttt

SEQ ID NO: 22 - DNA, 3252 bp, artificial
  Artificial
tcataagctttaatacgactcactataggcgtgtagttgtgctgcgtgtgtgaggagggctgagagagctcttttcgtatataaaggagggtacctataatctgtcctcctttatatacgaaaagagtatataaaggaggacaatatgcacatacaaagcttcgatcccgccgtcgttttacaacgtcgtgactgggaaaaccctggcgttacccaacttaatcgccttgcagcacatccccctttcgccagctggcgtaatagcgaagaggcccgcaccgatcgcccttcccaacagttgcgcagcctgaatggcgaatggcgctttgcctggtttccggcaccagaagcggtgccggaaagctggctggagtgcgatcttcctgaggccgatactgtcgtcgtcccctcaaactggcagatgcacggttacgatgcgcccatctacaccaacgtgacctatcccattacggtcaatccgccgtttgttcccacggagaatccgacgggttgttactcgctcacatttaatgttgatgaaagctggctacaggaaggccagacgcgaattatttttgatggcgttaactcggcgtttcatctgtggtgcaacgggcgctgggtcggttacggccaggacagtcgtttgccgtctgaatttgacctgagcgcatttttacgcgccggagaaaaccgcctcgcggtgatggtgctgcgctggagtgacggcagttatctggaagatcaggatatgtggcggatgagcggcattttccgtgacgtctcgttgctgcataaaccgactacacaaatcagcgatttccatgttgccactcgctttaatgatgatttcagccgcgctgtactggaggctgaagttcagatgtgcggcgagttgcgtgactacctacgggtaacagtttctttatggcagggtgaaacgcaggtcgccagcggcaccgcgcctttcggcggtgaaattatcgatgagcgtggtggttatgccgatcgcgtcacactacgtctgaacgtcgaaaacccgaaactgtggagcgccgaaatcccgaatctctatcgtgcggtggttgaactgcacaccgccgacggcacgctgattgaagcagaagcctgcgatgtcggtttccgcgaggtgcggattgaaaatggtctgctgctgctgaacggcaagccgttgctgattcgaggcgttaaccgtcacgagcatcatcctctgcatggtcaggtcatggatgagcagacgatggtgcaggatatcctgctgatgaagcagaacaactttaacgccgtgcgctgttcgcattatccgaaccatccgctgtggtacacgctgtgcgaccgctacggcctgtatgtggtggatgaagccaatattgaaacccacggcatggtgccaatgaatcgtctgaccgatgatccgcgctggctaccggcgatgagcgaacgcgtaacgcgaatggtgcagcgcgatcgtaatcacccgagtgtgatcatctggtcgctggggaatgaatcaggccacggcgctaatcacgacgcgctgtatcgctggatcaaatctgtcgatccttcccgcccggtgcagtatgaaggcggcggagccgacaccacggccaccgatattatttgcccgatgtacgcgcgcgtggatgaagaccagcccttcccggctgtgccgaaatggtccatcaaaaaatggctttcgctacctggagagacgcgcccgctgatcctttgcgaatacgcccacgcgatgggtaacagtcttggcggtttcgctaaatactggcaggcgtttcgtcagtatccccgtttacagggcggcttcgtctgggactgggtggatcagtcgctgattaaatatgatgaaaacggcaacccgtggtcggcttacggcggtgattttggcgatacgccgaacgatcgccagttctgtatgaacggtctggtctttgccgaccgcacgccgcatccagcgctgacggaagcaaaacaccagcagcagtttttccagttccgtttatccgggcaaaccatcgaagtgaccagcgaatacctgttccgtcatagcgataacgagctcctgcactggatggtggcgctggatggtaagccgctggcaagcggtgaagtgcctctggatgtcgctccacaaggtaaacagttgattgaactgcctgaactaccgcagccggagagcgccgggcaactctggctcacagtacgcgtagtgcaaccgaacgcgaccgcatggtcagaagccgggcacatcagcgcctggcagcagtggcgtctggcggaaaacctcagtgtgacgctccccgccgcgtcccacgccatcccgcatctgaccaccagcgaaatggatttttgcatcgagctgggtaataagcgttggcaatttaaccgccagtcaggctttctttcacagatgtggattggcgataaaaaacaactgctgacgccgctgcgcgatcagttcacccgtgcaccgctggataacgacattggcgtaagtgaagcgacccgcattgaccctaacgcctgggtcgaacgctggaaggcggcgggccattaccaggccgaagcagcgttgttgcagtgcacggcagatacacttgctgatgcggtgctgattacgaccgctcacgcgtggcagcatcaggggaaaaccttatttatcagccggaaaacctaccggattgatggtagtggtcaaatggcgattaccgttgatgttgaagtggcgagcgatacaccgcatccggcgcggattggcctgaactgccagctggcgcaggtagcagagcgggtaaactggctcggattagggccgcaagaaaactatcccgaccgccttactgccgcctgttttgaccgctgggatctgccattgtcagacatgtataccccgtacgtcttcccgagcgaaaacggtctgcgctgcgggacgcgcgaattgaattatggcccacaccagtggcgcggcgacttccagttcaacatcagccgctacagtcaacagcaactgatggaaaccagccatcgccatctgctgcacgcggaagaaggcacatggctgaatatcgacggtttccatatggggattggtggcgacgactcctggagcccgtcagtatcggcggaattccagctgagcgccggtcgctaccattaccagttggtctggtgtcaaaaataactagcataacccctctctaaacggaggggttt

SEQ ID NO: 23 - DNA, 759 bp, artificial
  Artificial
atgcgtaaaggagaagaacttttcactggagttgtcccaattcttgttgaattagatggtgatgttaatgggcacaaattttctgtcagtggagagggtgaaggtgatgcaacatacggaaaacttacccttaaatttatttgcactactggaaaactacctgttccgtggccaacacttgtcactactttcggttatggtgttcaatgctttgcgagatacccagatcacatgaaacagcatgactttttcaagagtgccatgcccgaaggttacgtacaggaaagaactatatttttcaaagatgacgggaactacaagacacgtgctgaagtcaagtttgaaggtgatacccttgttaatagaatcgagttaaaaggtattgattttaaagaagatggaaacattcttggacacaaattggaatacaactataactcacacaatgtatacatcatggcagacaaacaaaagaatggaatcaaagttaacttcaaaattagacacaacattgaagatggaagcgttcaactagcagaccattatcaacaaaatactccgattggcgatggccctgtccttttaccagacaaccattacctgtccacacaatctgccctttcgaaagatcccaacgaaaagagagaccacatggtccttcttgagtttgtaaccgctgctgggattacacatggcatggatgaactatacaaaaggcctgcagcaaacgacgaaaactacgctgcatcagtttaataa

SEQ ID NO: 24 - RNA, 167 nt, artificial
  Artificial
ggcguggcgaguuuggugcggucgugcugugugguaaauacguauaguacgaucggagggagggagaacaaucgguuuucuccuuuugaucguauuauacgaucaaaaggaggagauaauguacauuugcaaccuggcggcagcgcaaaagaugcguaaaggagaag

SEQ ID NO: 25 - RNA, 167 nt, artificial
  Artificial
ggcguguagcuauguugcguguauggggagggcgaaaaucgcuuuucucguauauaaaggagggagcacuuaauacuuccuccuuuauauacgagaaggguauauaaaggaggaagcaauggaaguuggcaaccuggcggcagcgcaaaagaugcguaaaggagaag

SEQ ID NO: 26 - RNA, 167 nt, artificial
  Artificial
ggcguguggaggagguuuucggguuguaaaguaauacauuuauuuugcgauucgauagggaggaaguacacauaucuuccuccuuauuggaucgcgagauaucaauaaggaggaagaaaugcaaauugcgaaccuggcggcagcgcaaaagaugcguaaaggagaag

SEQ ID NO: 27 - DNA, 1105 bp, artificial
  Artificial
ggcaacagatctcacagctaacaccacgtcgtccctatctgctgccctaggtctatgagtggttgctggataactttacgggcatgcataaggctcgtataatatattcaagtaatactggaagcaatgtgagcaatgtcgtgctgttatagttatgagacaagaacagaggagacataacatgaacagcacgaacgctgttaacctggcggcagcgcaaaagatgcgtaaaggagaagaacttttcactggagttgtcccaattcttgttgaattagatggtgatgttaatgggcacaaattttctgtcagtggagagggtgaaggtgatgcaacatacggaaaacttacccttaaatttatttgcactactggaaaactacctgttccgtggccaacacttgtcactactttcggttatggtgttcaatgctttgcgagatacccagatcacatgaaacagcatgactttttcaagagtgccatgcccgaaggttacgtacaggaaagaactatatttttcaaagatgacgggaactacaagacacgtgctgaagtcaagtttgaaggtgatacccttgttaatagaatcgagttaaaaggtattgattttaaagaagatggaaacattcttggacacaaattggaatacaactataactcacacaatgtatacatcatggcagacaaacaaaagaatggaatcaaagttaacttcaaaattagacacaacattgaagatggaagcgttcaactagcagaccattatcaacaaaatactccgattggcgatggccctgtccttttaccagacaaccattacctgtccacacaatctgccctttcgaaagatcccaacgaaaagagagaccacatggtccttcttgagtttgtaaccgctgctgggattacacatggcatggatgaactatacaaaaggcctgcagcaaacgacgaaaactacgctgcatcagtttaataagataaaccagagcggcacggcaagcagagtatacgagattcggtagccaccgctgagcaataactagcataaccccttggggcctctaaacgggtcttgaggggttttttgcatatgcaacgg

SEQ ID NO: 28 - DNA, 43 bp, artificial
  Artificial
ccgttgcatatgcaaaaaacccctcaagacccgtttagaggcc

SEQ ID NO: 29 - DNA, 194 bp, artificial
  Artificial
tcataagctttaatacgactcactataggcgtggcgagtttggtgcggtcgtgctgtgtggtaaatacgtatagtacgatcggagggagggagaacaatcggttttctccttttgatcgtattatacgatcaaaaggaggagataatgtacatttgcaacctggcggcagcgcaaaagatgcgtaaaggagaag

SEQ ID NO: 30 - DNA, 194 bp, artificial
  Artificial
tcataagctttaatacgactcactataggcgtgtagctatgttgcgtgtatggggagggcgaaaatcgcttttctcgtatataaaggagggagcacttaatacttcctcctttatatacgagaagggtatataaaggaggaagcaatggaagttggcaacctggcggcagcgcaaaagatgcgtaaaggagaag

SEQ ID NO: 31 - DNA, 194 bp, artificial
  Artificial
tcataagctttaatacgactcactataggcgtgtggaggaggttttcgggttgtaaagtaatacatttattttgcgattcgatagggaggaagtacacatatcttcctccttattggatcgcgagatatcaataaggaggaagaaatgcaaattgcgaacctggcggcagcgcaaaagatgcgtaaaggagaag

SEQ ID NO: 32 - DNA, 1063 bp, artificial
  Artificial
tcataagctttaatacgactcactataggcgtggcgagtttggtgcggtcgtgctgtgtggtaaatacgtatagtacgatcggagggagggagaacaatcggttttctccttttgatcgtattatacgatcaaaaggaggagataatgtacatttgcaacctggcggcagcgcaaaagatgcgtaaaggagaagaacttttcactggagttgtcccaattcttgttgaattagatggtgatgttaatgggcacaaattttctgtcagtggagagggtgaaggtgatgcaacatacggaaaacttacccttaaatttatttgcactactggaaaactacctgttccgtggccaacacttgtcactactttcggttatggtgttcaatgctttgcgagatacccagatcacatgaaacagcatgactttttcaagagtgccatgcccgaaggttacgtacaggaaagaactatatttttcaaagatgacgggaactacaagacacgtgctgaagtcaagtttgaaggtgatacccttgttaatagaatcgagttaaaaggtattgattttaaagaagatggaaacattcttggacacaaattggaatacaactataactcacacaatgtatacatcatggcagacaaacaaaagaatggaatcaaagttaacttcaaaattagacacaacattgaagatggaagcgttcaactagcagaccattatcaacaaaatactccgattggcgatggccctgtccttttaccagacaaccattacctgtccacacaatctgccctttcgaaagatcccaacgaaaagagagaccacatggtccttcttgagtttgtaaccgctgctgggattacacatggcatggatgaactatacaaaaggcctgcagcaaacgacgaaaactacgctgcatcagtttaataataagataaaccagagcggcacggcaagcagagtatacgagattcggtagccaccgctgagcaataactagcataaccccttggggcctctaaacgggtcttgaggggttttttgcatatgcaacgg

SEQ ID NO: 33 - DNA, 1063 bp, artificial
  Artificial
tcataagctttaatacgactcactataggcgtgtagctatgttgcgtgtatggggagggcgaaaatcgcttttctcgtatataaaggagggagcacttaatacttcctcctttatatacgagaagggtatataaaggaggaagcaatggaagttggcaacctggcggcagcgcaaaagatgcgtaaaggagaagaacttttcactggagttgtcccaattcttgttgaattagatggtgatgttaatgggcacaaattttctgtcagtggagagggtgaaggtgatgcaacatacggaaaacttacccttaaatttatttgcactactggaaaactacctgttccgtggccaacacttgtcactactttcggttatggtgttcaatgctttgcgagatacccagatcacatgaaacagcatgactttttcaagagtgccatgcccgaaggttacgtacaggaaagaactatatttttcaaagatgacgggaactacaagacacgtgctgaagtcaagtttgaaggtgatacccttgttaatagaatcgagttaaaaggtattgattttaaagaagatggaaacattcttggacacaaattggaatacaactataactcacacaatgtatacatcatggcagacaaacaaaagaatggaatcaaagttaacttcaaaattagacacaacattgaagatggaagcgttcaactagcagaccattatcaacaaaatactccgattggcgatggccctgtccttttaccagacaaccattacctgtccacacaatctgccctttcgaaagatcccaacgaaaagagagaccacatggtccttcttgagtttgtaaccgctgctgggattacacatggcatggatgaactatacaaaaggcctgcagcaaacgacgaaaactacgctgcatcagtttaataataagataaaccagagcggcacggcaagcagagtatacgagattcggtagccaccgctgagcaataactagcataaccccttggggcctctaaacgggtcttgaggggttttttgcatatgcaacgg

SEQ ID NO: 34 - DNA, 1063 bp, artificial
  Artificial
tcataagctttaatacgactcactataggcgtgtggaggaggttttcgggttgtaaagtaatacatttattttgcgattcgatagggaggaagtacacatatcttcctccttattggatcgcgagatatcaataaggaggaagaaatgcaaattgcgaacctggcggcagcgcaaaagatgcgtaaaggagaagaacttttcactggagttgtcccaattcttgttgaattagatggtgatgttaatgggcacaaattttctgtcagtggagagggtgaaggtgatgcaacatacggaaaacttacccttaaatttatttgcactactggaaaactacctgttccgtggccaacacttgtcactactttcggttatggtgttcaatgctttgcgagatacccagatcacatgaaacagcatgactttttcaagagtgccatgcccgaaggttacgtacaggaaagaactatatttttcaaagatgacgggaactacaagacacgtgctgaagtcaagtttgaaggtgatacccttgttaatagaatcgagttaaaaggtattgattttaaagaagatggaaacattcttggacacaaattggaatacaactataactcacacaatgtatacatcatggcagacaaacaaaagaatggaatcaaagttaacttcaaaattagacacaacattgaagatggaagcgttcaactagcagaccattatcaacaaaatactccgattggcgatggccctgtccttttaccagacaaccattacctgtccacacaatctgccctttcgaaagatcccaacgaaaagagagaccacatggtccttcttgagtttgtaaccgctgctgggattacacatggcatggatgaactatacaaaaggcctgcagcaaacgacgaaaactacgctgcatcagtttaataataagataaaccagagcggcacggcaagcagagtatacgagattcggtagccaccgctgagcaataactagcataaccccttggggcctctaaacgggtcttgaggggttttttgcatatgcaacgg

SEQ ID NO: 35 - DNA, 21290 bp, severe acute respiratory syndrome coronavirus 2 isolate wuhan-hu-1 (sars-cov-2)
atggagagccttgtccctggtttcaacgagaaaacacacgtccaactcagtttgcctgttttacaggttcgcgacgtgctcgtacgtggctttggagactccgtggaggaggtcttatcagaggcacgtcaacatcttaaagatggcacttgtggcttagtagaagttgaaaaaggcgttttgcctcaacttgaacagccctatgtgttcatcaaacgttcggatgctcgaactgcacctcatggtcatgttatggttgagctggtagcagaactcgaaggcattcagtacggtcgtagtggtgagacacttggtgtccttgtccctcatgtgggcgaaataccagtggcttaccgcaaggttcttcttcgtaagaacggtaataaaggagctggtggccatagttacggcgccgatctaaagtcatttgacttaggcgacgagcttggcactgatccttatgaagattttcaagaaaactggaacactaaacatagcagtggtgttacccgtgaactcatgcgtgagcttaacggaggggcatacactcgctatgtcgataacaacttctgtggccctgatggctaccctcttgagtgcattaaagaccttctagcacgtgctggtaaagcttcatgcactttgtccgaacaactggactttattgacactaagaggggtgtatactgctgccgtgaacatgagcatgaaattgcttggtacacggaacgttctgaaaagagctatgaattgcagacaccttttgaaattaaattggcaaagaaatttgacaccttcaatggggaatgtccaaattttgtatttcccttaaattccataatcaagactattcaaccaagggttgaaaagaaaaagcttgatggctttatgggtagaattcgatctgtctatccagttgcgtcaccaaatgaatgcaaccaaatgtgcctttcaactctcatgaagtgtgatcattgtggtgaaacttcatggcagacgggcgattttgttaaagccacttgcgaattttgtggcactgagaatttgactaaagaaggtgccactacttgtggttacttaccccaaaatgctgttgttaaaatttattgtccagcatgtcacaattcagaagtaggacctgagcatagtcttgccgaataccataatgaatctggcttgaaaaccattcttcgtaagggtggtcgcactattgcctttggaggctgtgtgttctcttatgttggttgccataacaagtgtgcctattgggttccacgtgctagcgctaacataggttgtaaccatacaggtgttgttggagaaggttccgaaggtcttaatgacaaccttcttgaaatactccaaaaagagaaagtcaacatcaatattgttggtgactttaaacttaatgaagagatcgccattattttggcatctttttctgcttccacaagtgcttttgtggaaactgtgaaaggtttggattataaagcattcaaacaaattgttgaatcctgtggtaattttaaagttacaaaaggaaaagctaaaaaaggtgcctggaatattggtgaacagaaatcaatactgagtcctctttatgcatttgcatcagaggctgctcgtgttgtacgatcaattttctcccgcactcttgaaactgctcaaaattctgtgcgtgttttacagaaggccgctataacaatactagatggaatttcacagtattcactgagactcattgatgctatgatgttcacatctgatttggctactaacaatctagttgtaatggcctacattacaggtggtgttgttcagttgacttcgcagtggctaactaacatctttggcactgtttatgaaaaactcaaacccgtccttgattggcttgaagagaagtttaaggaaggtgtagagtttcttagagacggttgggaaattgttaaatttatctcaacctgtgcttgtgaaattgtcggtggacaaattgtcacctgtgcaaaggaaattaaggagagtgttcagacattctttaagcttgtaaataaatttttggctttgtgtgctgactctatcattattggtggagctaaacttaaagccttgaatttaggtgaaacatttgtcacgcactcaaagggattgtacagaaagtgtgttaaatccagagaagaaactggcctactcatgcctctaaaagccccaaaagaaattatcttcttagagggagaaacacttcccacagaagtgttaacagaggaagttgtcttgaaaactggtgatttacaaccattagaacaacctactagtgaagctgttgaagctccattggttggtacaccagtttgtattaacgggcttatgttgctcgaaatcaaagacacagaaaagtactgtgcccttgcacctaatatgatggtaacaaacaataccttcacactcaaaggcggtgcaccaacaaaggttacttttggtgatgacactgtgatagaagtgcaaggttacaagagtgtgaatatcacttttgaacttgatgaaaggattgataaagtacttaatgagaagtgctctgcctatacagttgaactcggtacagaagtaaatgagttcgcctgtgttgtggcagatgctgtcataaaaactttgcaaccagtatctgaattacttacaccactgggcattgatttagatgagtggagtatggctacatactacttatttgatgagtctggtgagtttaaattggcttcacatatgtattgttctttctaccctccagatgaggatgaagaagaaggtgattgtgaagaagaagagtttgagccatcaactcaatatgagtatggtactgaagatgattaccaaggtaaacctttggaatttggtgccacttctgctgctcttcaacctgaagaagagcaagaagaagattggttagatgatgatagtcaacaaactgttggtcaacaagacggcagtgaggacaatcagacaactactattcaaacaattgttgaggttcaacctcaattagagatggaacttacaccagttgttcagactattgaagtgaatagttttagtggttatttaaaacttactgacaatgtatacattaaaaatgcagacattgtggaagaagctaaaaaggtaaaaccaacagtggttgttaatgcagccaatgtttaccttaaacatggaggaggtgttgcaggagccttaaataaggctactaacaatgccatgcaagttgaatctgatgattacatagctactaatggaccacttaaagtgggtggtagttgtgttttaagcggacacaatcttgctaaacactgtcttcatgttgtcggcccaaatgttaacaaaggtgaagacattcaacttcttaagagtgcttatgaaaattttaatcagcacgaagttctacttgcaccattattatcagctggtatttttggtgctgaccctatacattctttaagagtttgtgtagatactgttcgcacaaatgtctacttagctgtctttgataaaaatctctatgacaaacttgtttcaagctttttggaaatgaagagtgaaaagcaagttgaacaaaagatcgctgagattcctaaagaggaagttaagccatttataactgaaagtaaaccttcagttgaacagagaaaacaagatgataagaaaatcaaagcttgtgttgaagaagttacaacaactctggaagaaactaagttcctcacagaaaacttgttactttatattgacattaatggcaatcttcatccagattctgccactcttgttagtgacattgacatcactttcttaaagaaagatgctccatatatagtgggtgatgttgttcaagagggtgttttaactgctgtggttatacctactaaaaaggctggtggcactactgaaatgctagcgaaagctttgagaaaagtgccaacagacaattatataaccacttacccgggtcagggtttaaatggttacactgtagaggaggcaaagacagtgcttaaaaagtgtaaaagtgccttttacattctaccatctattatctctaatgagaagcaagaaattcttggaactgtttcttggaatttgcgagaaatgcttgcacatgcagaagaaacacgcaaattaatgcctgtctgtgtggaaactaaagccatagtttcaactatacagcgtaaatataagggtattaaaatacaagagggtgtggttgattatggtgctagattttacttttacaccagtaaaacaactgtagcgtcacttatcaacacacttaacgatctaaatgaaactcttgttacaatgccacttggctatgtaacacatggcttaaatttggaagaagctgctcggtatatgagatctctcaaagtgccagctacagtttctgtttcttcacctgatgctgttacagcgtataatggttatcttacttcttcttctaaaacacctgaagaacattttattgaaaccatctcacttgctggttcctataaagattggtcctattctggacaatctacacaactaggtatagaatttcttaagagaggtgataaaagtgtatattacactagtaatcctaccacattccacctagatggtgaagttatcacctttgacaatcttaagacacttctttctttgagagaagtgaggactattaaggtgtttacaacagtagacaacattaacctccacacgcaagttgtggacatgtcaatgacatatggacaacagtttggtccaacttatttggatggagctgatgttactaaaataaaacctcataattcacatgaaggtaaaacattttatgttttacctaatgatgacactctacgtgttgaggcttttgagtactaccacacaactgatcctagttttctgggtaggtacatgtcagcattaaatcacactaaaaagtggaaatacccacaagttaatggtttaacttctattaaatgggcagataacaactgttatcttgccactgcattgttaacactccaacaaatagagttgaagtttaatccacctgctctacaagatgcttattacagagcaagggctggtgaagctgctaacttttgtgcacttatcttagcctactgtaataagacagtaggtgagttaggtgatgttagagaaacaatgagttacttgtttcaacatgccaatttagattcttgcaaaagagtcttgaacgtggtgtgtaaaacttgtggacaacagcagacaacccttaagggtgtagaagctgttatgtacatgggcacactttcttatgaacaatttaagaaaggtgttcagataccttgtacgtgtggtaaacaagctacaaaatatctagtacaacaggagtcaccttttgttatgatgtcagcaccacctgctcagtatgaacttaagcatggtacatttacttgtgctagtgagtacactggtaattaccagtgtggtcactataaacatataacttctaaagaaactttgtattgcatagacggtgctttacttacaaagtcctcagaatacaaaggtcctattacggatgttttctacaaagaaaacagttacacaacaaccataaaaccagttacttataaattggatggtgttgtttgtacagaaattgaccctaagttggacaattattataagaaagacaattcttatttcacagagcaaccaattgatcttgtaccaaaccaaccatatccaaacgcaagcttcgataattttaagtttgtatgtgataatatcaaatttgctgatgatttaaaccagttaactggttataagaaacctgcttcaagagagcttaaagttacatttttccctgacttaaatggtgatgtggtggctattgattataaacactacacaccctcttttaagaaaggagctaaattgttacataaacctattgtttggcatgttaacaatgcaactaataaagccacgtataaaccaaatacctggtgtatacgttgtctttggagcacaaaaccagttgaaacatcaaattcgtttgatgtactgaagtcagaggacgcgcagggaatggataatcttgcctgcgaagatctaaaaccagtctctgaagaagtagtggaaaatcctaccatacagaaagacgttcttgagtgtaatgtgaaaactaccgaagttgtaggagacattatacttaaaccagcaaataatagtttaaaaattacagaagaggttggccacacagatctaatggctgcttatgtagacaattctagtcttactattaagaaacctaatgaattatctagagtattaggtttgaaaacccttgctactcatggtttagctgctgttaatagtgtcccttgggatactatagctaattatgctaagccttttcttaacaaagttgttagtacaactactaacatagttacacggtgtttaaaccgtgtttgtactaattatatgccttatttctttactttattgctacaattgtgtacttttactagaagtacaaattctagaattaaagcatctatgccgactactatagcaaagaatactgttaagagtgtcggtaaattttgtctagaggcttcatttaattatttgaagtcacctaatttttctaaactgataaatattataatttggtttttactattaagtgtttgcctaggttctttaatctactcaaccgctgctttaggtgttttaatgtctaatttaggcatgccttcttactgtactggttacagagaaggctatttgaactctactaatgtcactattgcaacctactgtactggttctataccttgtagtgtttgtcttagtggtttagattctttagacacctatccttctttagaaactatacaaattaccatttcatcttttaaatgggatttaactgcttttggcttagttgcagagtggtttttggcatatattcttttcactaggtttttctatgtacttggattggctgcaatcatgcaattgtttttcagctattttgcagtacattttattagtaattcttggcttatgtggttaataattaatcttgtacaaatggccccgatttcagctatggttagaatgtacatcttctttgcatcattttattatgtatggaaaagttatgtgcatgttgtagacggttgtaattcatcaacttgtatgatgtgttacaaacgtaatagagcaacaagagtcgaatgtacaactattgttaatggtgttagaaggtccttttatgtctatgctaatggaggtaaaggcttttgcaaactacacaattggaattgtgttaattgtgatacattctgtgctggtagtacatttattagtgatgaagttgcgagagacttgtcactacagtttaaaagaccaataaatcctactgaccagtcttcttacatcgttgatagtgttacagtgaagaatggttccatccatctttactttgataaagctggtcaaaagacttatgaaagacattctctctctcattttgttaacttagacaacctgagagctaataacactaaaggttcattgcctattaatgttatagtttttgatggtaaatcaaaatgtgaagaatcatctgcaaaatcagcgtctgtttactacagtcagcttatgtgtcaacctatactgttactagatcaggcattagtgtctgatgttggtgatagtgcggaagttgcagttaaaatgtttgatgcttacgttaatacgttttcatcaacttttaacgtaccaatggaaaaactcaaaacactagttgcaactgcagaagctgaacttgcaaagaatgtgtccttagacaatgtcttatctacttttatttcagcagctcggcaagggtttgttgattcagatgtagaaactaaagatgttgttgaatgtcttaaattgtcacatcaatctgacatagaagttactggcgatagttgtaataactatatgctcacctataacaaagttgaaaacatgacaccccgtgaccttggtgcttgtattgactgtagtgcgcgtcatattaatgcgcaggtagcaaaaagtcacaacattgctttgatatggaacgttaaagatttcatgtcattgtctgaacaactacgaaaacaaatacgtagtgctgctaaaaagaataacttaccttttaagttgacatgtgcaactactagacaagttgttaatgttgtaacaacaaagatagcacttaagggtggtaaaattgttaataattggttgaagcagttaattaaagttacacttgtgttcctttttgttgctgctattttctatttaataacacctgttcatgtcatgtctaaacatactgacttttcaagtgaaatcataggatacaaggctattgatggtggtgtcactcgtgacatagcatctacagatacttgttttgctaacaaacatgctgattttgacacatggtttagccagcgtggtggtagttatactaatgacaaagcttgcccattgattgctgcagtcataacaagagaagtgggttttgtcgtgcctggtttgcctggcacgatattacgcacaactaatggtgactttttgcatttcttacctagagtttttagtgcagttggtaacatctgttacacaccatcaaaacttatagagtacactgactttgcaacatcagcttgtgttttggctgctgaatgtacaatttttaaagatgcttctggtaagccagtaccatattgttatgataccaatgtactagaaggttctgttgcttatgaaagtttacgccctgacacacgttatgtgctcatggatggctctattattcaatttcctaacacctaccttgaaggttctgttagagtggtaacaacttttgattctgagtactgtaggcacggcacttgtgaaagatcagaagctggtgtttgtgtatctactagtggtagatgggtacttaacaatgattattacagatctttaccaggagttttctgtggtgtagatgctgtaaatttacttactaatatgtttacaccactaattcaacctattggtgctttggacatatcagcatctatagtagctggtggtattgtagctatcgtagtaacatgccttgcctactattttatgaggtttagaagagcttttggtgaatacagtcatgtagttgcctttaatactttactattccttatgtcattcactgtactctgtttaacaccagtttactcattcttacctggtgtttattctgttatttacttgtacttgacattttatcttactaatgatgtttcttttttagcacatattcagtggatggttatgttcacacctttagtacctttctggataacaattgcttatatcatttgtatttccacaaagcatttctattggttctttagtaattacctaaagagacgtgtagtctttaatggtgtttcctttagtacttttgaagaagctgcgctgtgcacctttttgttaaataaagaaatgtatctaaagttgcgtagtgatgtgctattacctcttacgcaatataatagatacttagctctttataataagtacaagtattttagtggagcaatggatacaactagctacagagaagctgcttgttgtcatctcgcaaaggctctcaatgacttcagtaactcaggttctgatgttctttaccaaccaccacaaacctctatcacctcagctgttttgcagagtggttttagaaaaatggcattcccatctggtaaagttgagggttgtatggtacaagtaacttgtggtacaactacacttaacggtctttggcttgatgacgtagtttactgtccaagacatgtgatctgcacctctgaagacatgcttaaccctaattatgaagatttactcattcgtaagtctaatcataatttcttggtacaggctggtaatgttcaactcagggttattggacattctatgcaaaattgtgtacttaagcttaaggttgatacagccaatcctaagacacctaagtataagtttgttcgcattcaaccaggacagactttttcagtgttagcttgttacaatggttcaccatctggtgtttaccaatgtgctatgaggcccaatttcactattaagggttcattccttaatggttcatgtggtagtgttggttttaacatagattatgactgtgtctctttttgttacatgcaccatatggaattaccaactggagttcatgctggcacagacttagaaggtaacttttatggaccttttgttgacaggcaaacagcacaagcagctggtacggacacaactattacagttaatgttttagcttggttgtacgctgctgttataaatggagacaggtggtttctcaatcgatttaccacaactcttaatgactttaaccttgtggctatgaagtacaattatgaacctctaacacaagaccatgttgacatactaggacctctttctgctcaaactggaattgccgttttagatatgtgtgcttcattaaaagaattactgcaaaatggtatgaatggacgtaccatattgggtagtgctttattagaagatgaatttacaccttttgatgttgttagacaatgctcaggtgttactttccaaagtgcagtgaaaagaacaatcaagggtacacaccactggttgttactcacaattttgacttcacttttagttttagtccagagtactcaatggtctttgttcttttttttgtatgaaaatgcctttttaccttttgctatgggtattattgctatgtctgcttttgcaatgatgtttgtcaaacataagcatgcatttctctgtttgtttttgttaccttctcttgccactgtagcttattttaatatggtctatatgcctgctagttgggtgatgcgtattatgacatggttggatatggttgatactagtttgtctggttttaagctaaaagactgtgttatgtatgcatcagctgtagtgttactaatccttatgacagcaagaactgtgtatgatgatggtgctaggagagtgtggacacttatgaatgtcttgacactcgtttataaagtttattatggtaatgctttagatcaagccatttccatgtgggctcttataatctctgttacttctaactactcaggtgtagttacaactgtcatgtttttggccagaggtattgtttttatgtgtgttgagtattgccctattttcttcataactggtaatacacttcagtgtataatgctagtttattgtttcttaggctatttttgtacttgttactttggcctcttttgtttactcaaccgctactttagactgactcttggtgtttatgattacttagtttctacacaggagtttagatatatgaattcacagggactactcccacccaagaatagcatagatgccttcaaactcaacattaaattgttgggtgttggtggcaaaccttgtatcaaagtagccactgtacagtctaaaatgtcagatgtaaagtgcacatcagtagtcttactctcagttttgcaacaactcagagtagaatcatcatctaaattgtgggctcaatgtgtccagttacacaatgacattctcttagctaaagatactactgaagcctttgaaaaaatggtttcactactttctgttttgctttccatgcagggtgctgtagacataaacaagctttgtgaagaaatgctggacaacagggcaaccttacaagctatagcctcagagtttagttcccttccatcatatgcagcttttgctactgctcaagaagcttatgagcaggctgttgctaatggtgattctgaagttgttcttaaaaagttgaagaagtctttgaatgtggctaaatctgaatttgaccgtgatgcagccatgcaacgtaagttggaaaagatggctgatcaagctatgacccaaatgtataaacaggctagatctgaggacaagagggcaaaagttactagtgctatgcagacaatgcttttcactatgcttagaaagttggataatgatgcactcaacaacattatcaacaatgcaagagatggttgtgttcccttgaacataatacctcttacaacagcagccaaactaatggttgtcataccagactataacacatataaaaatacgtgtgatggtacaacatttacttatgcatcagcattgtgggaaatccaacaggttgtagatgcagatagtaaaattgttcaacttagtgaaattagtatggacaattcacctaatttagcatggcctcttattgtaacagctttaagggccaattctgctgtcaaattacagaataatgagcttagtcctgttgcactacgacagatgtcttgtgctgccggtactacacaaactgcttgcactgatgacaatgcgttagcttactacaacacaacaaagggaggtaggtttgtacttgcactgttatccgatttacaggatttgaaatgggctagattccctaagagtgatggaactggtactatctatacagaactggaaccaccttgtaggtttgttacagacacacctaaaggtcctaaagtgaagtatttatactttattaaaggattaaacaacctaaatagaggtatggtacttggtagtttagctgccacagtacgtctacaagctggtaatgcaacagaagtgcctgccaattcaactgtattatctttctgtgcttttgctgtagatgctgctaaagcttacaaagattatctagctagtgggggacaaccaatcactaattgtgttaagatgttgtgtacacacactggtactggtcaggcaataacagttacaccggaagccaatatggatcaagaatcctttggtggtgcatcgtgttgtctgtactgccgttgccacatagatcatccaaatcctaaaggattttgtgacttaaaaggtaagtatgtacaaatacctacaacttgtgctaatgaccctgtgggttttacacttaaaaacacagtctgtaccgtctgcggtatgtggaaaggttatggctgtagttgtgatcaactccgcgaacccatgcttcagtcagctgatgcacaatcgtttttaaacgggtttgcggtgtaagtgcagcccgtcttacaccgtgcggcacaggcactagtactgatgtcgtatacagggcttttgacatctacaatgataaagtagctggttttgctaaattcctaaaaactaattgttgtcgcttccaagaaaaggacgaagatgacaatttaattgattcttactttgtagttaagagacacactttctctaactaccaacatgaagaaacaatttataatttacttaaggattgtccagctgttgctaaacatgacttctttaagtttagaatagacggtgacatggtaccacatatatcacgtcaacgtcttactaaatacacaatggcagacctcgtctatgctttaaggcattttgatgaaggtaattgtgacacattaaaagaaatacttgtcacatacaattgttgtgatgatgattatttcaataaaaaggactggtatgattttgtagaaaacccagatatattacgcgtatacgccaacttaggtgaacgtgtacgccaagctttgttaaaaacagtacaattctgtgatgccatgcgaaatgctggtattgttggtgtactgacattagataatcaagatctcaatggtaactggtatgatttcggtgatttcatacaaaccacgccaggtagtggagttcctgttgtagattcttattattcattgttaatgcctatattaaccttgaccagggctttaactgcagagtcacatgttgacactgacttaacaaagccttacattaagtgggatttgttaaaatatgacttcacggaagagaggttaaaactctttgaccgttattttaaatattgggatcagacataccacccaaattgtgttaactgtttggatgacagatgcattctgcattgtgcaaactttaatgttttattctctacagtgttcccacctacaagttttggaccactagtgagaaaaatatttgttgatggtgttccatttgtagtttcaactggataccacttcagagagctaggtgttgtacataatcaggatgtaaacttacatagctctagacttagttttaaggaattacttgtgtatgctgctgaccctgctatgcacgctgcttctggtaatctattactagataaacgcactacgtgcttttcagtagctgcacttactaacaatgttgcttttcaaactgtcaaacccggtaattttaacaaagacttctatgactttgctgtgtctaagggtttctttaaggaaggaagttctgttgaattaaaacacttcttctttgctcaggatggtaatgctgctatcagcgattatgactactatcgttataatctaccaacaatgtgtgatatcagacaactactatttgtagttgaagttgttgataagtactttgattgttacgatggtggctgtattaatgctaaccaagtcatcgtcaacaacctagacaaatcagctggttttccatttaataaatggggtaaggctagactttattatgattcaatgagttatgaggatcaagatgcacttttcgcatatacaaaacgtaatgtcatccctactataactcaaatgaatcttaagtatgccattagtgcaaagaatagagctcgcaccgtagctggtgtctctatctgtagtactatgaccaatagacagtttcatcaaaaattattgaaatcaatagccgccactagaggagctactgtagtaattggaacaagcaaattctatggtggttggcacaacatgttaaaaactgtttatagtgatgtagaaaaccctcaccttatgggttgggattatcctaaatgtgatagagccatgcctaacatgcttagaattatggcctcacttgttcttgctcgcaaacatacaacgtgttgtagcttgtcacaccgtttctatagattagctaatgagtgtgctcaagtattgagtgaaatggtcatgtgtggcggttcactatatgttaaaccaggtggaacctcatcaggagatgccacaactgcttatgctaatagtgtttttaacatttgtcaagctgtcacggccaatgttaatgcacttttatctactgatggtaacaaaattgccgataagtatgtccgcaatttacaacacagactttatgagtgtctctatagaaatagagatgttgacacagactttgtgaatgagttttacgcatatttgcgtaaacatttctcaatgatgatactctctgacgatgctgttgtgtgtttcaatagcacttatgcatctcaaggtctagtggctagcataaagaactttaagtcagttctttattatcaaaacaatgtttttatgtctgaagcaaaatgttggactgagactgaccttactaaaggacctcatgaattttgctctcaacatacaatgctagttaaacagggtgatgattatgtgtaccttccttacccagatccatcaagaatcctaggggccggctgttttgtagatgatatcgtaaaaacagatggtacacttatgattgaacggttcgtgtctttagctatagatgcttacccacttactaaacatcctaatcaggagtatgctgatgtctttcatttgtacttacaatacataagaaagctacatgatgagttaacaggacacatgttagacatgtattctgttatgcttactaatgataacacttcaaggtattgggaacctgagttttatgaggctatgtacacaccgcatacagtcttacaggctgttggggcttgtgttctttgcaattcacagacttcattaagatgtggtgcttgcatacgtagaccattcttatgttgtaaatgctgttacgaccatgtcatatcaacatcacataaattagtcttgtctgttaatccgtatgtttgcaatgctccaggttgtgatgtcacagatgtgactcaactttacttaggaggtatgagctattattgtaaatcacataaaccacccattagttttccattgtgtgctaatggacaagtttttggtttatataaaaatacatgtgttggtagcgataatgttactgactttaatgcaattgcaacatgtgactggacaaatgctggtgattacattttagctaacacctgtactgaaagactcaagctttttgcagcagaaacgctcaaagctactgaggagacatttaaactgtcttatggtattgctactgtacgtgaagtgctgtctgacagagaattacatctttcatgggaagttggtaaacctagaccaccacttaaccgaaattatgtctttactggttatcgtgtaactaaaaacagtaaagtacaaataggagagtacacctttgaaaaaggtgactatggtgatgctgttgtttaccgaggtacaacaacttacaaattaaatgttggtgattattttgtgctgacatcacatacagtaatgccattaagtgcacctacactagtgccacaagagcactatgttagaattactggcttatacccaacactcaatatctcagatgagttttctagcaatgttgcaaattatcaaaaggttggtatgcaaaagtattctacactccagggaccacctggtactggtaagagtcattttgctattggcctagctctctactacccttctgctcgcatagtgtatacagcttgctctcatgccgctgttgatgcactatgtgagaaggcattaaaatatttgcctatagataaatgtagtagaattatacctgcacgtgctcgtgtagagtgttttgataaattcaaagtgaattcaacattagaacagtatgtcttttgtactgtaaatgcattgcctgagacgacagcagatatagttgtctttgatgaaatttcaatggccacaaattatgatttgagtgttgtcaatgccagattacgtgctaagcactatgtgtacattggcgaccctgctcaattacctgcaccacgcacattgctaactaagggcacactagaaccagaatatttcaattcagtgtgtagacttatgaaaactataggtccagacatgttcctcggaacttgtcggcgttgtcctgctgaaattgttgacactgtgagtgctttggtttatgataataagcttaaagcacataaagacaaatcagctcaatgctttaaaatgttttataagggtgttatcacgcatgatgtttcatctgcaattaacaggccacaaataggcgtggtaagagaattccttacacgtaaccctgcttggagaaaagctgtctttatttcaccttataattcacagaatgctgtagcctcaaagattttgggactaccaactcaaactgttgattcatcacagggctcagaatatgactatgtcatattcactcaaaccactgaaacagctcactcttgtaatgtaaacagatttaatgttgctattaccagagcaaaagtaggcatactttgcataatgtctgatagagacctttatgacaagttgcaatttacaagtcttgaaattccacgtaggaatgtggcaactttacaagctgaaaatgtaacaggactctttaaagattgtagtaaggtaatcactgggttacatcctacacaggcacctacacacctcagtgttgacactaaattcaaaactgaaggtttatgtgttgacatacctggcatacctaaggacatgacctatagaagactcatctctatgatgggttttaaaatgaattatcaagttaatggttaccctaacatgtttatcacccgcgaagaagctataagacatgtacgtgcatggattggcttcgatgtcgaggggtgtcatgctactagagaagctgttggtaccaatttacctttacagctaggtttttctacaggtgttaacctagttgctgtacctacaggttatgttgatacacctaataatacagatttttccagagttagtgctaaaccaccgcctggagatcaatttaaacacctcataccacttatgtacaaaggacttccttggaatgtagtgcgtataaagattgtacaaatgttaagtgacacacttaaaaatctctctgacagagtcgtatttgtcttatgggcacatggctttgagttgacatctatgaagtattttgtgaaaataggacctgagcgcacctgttgtctatgtgatagacgtgccacatgcttttccactgcttcagacacttatgcctgttggcatcattctattggatttgattacgtctataatccgtttatgattgatgttcaacaatggggttttacaggtaacctacaaagcaaccatgatctgtattgtcaagtccatggtaatgcacatgtagctagttgtgatgcaatcatgactaggtgtctagctgtccacgagtgctttgttaagcgtgttgactggactattgaatatcctataattggtgatgaactgaagattaatgcggcttgtagaaaggttcaacacatggttgttaaagctgcattattagcagacaaattcccagttcttcacgacattggtaaccctaaagctattaagtgtgtacctcaagctgatgtagaatggaagttctatgatgcacagccttgtagtgacaaagcttataaaatagaagaattattctattcttatgccacacattctgacaaattcacagatggtgtatgcctattttggaattgcaatgtcgatagatatcctgctaattccattgtttgtagatttgacactagagtgctatctaaccttaacttgcctggttgtgatggtggcagtttgtatgtaaataaacatgcattccacacaccagcttttgataaaagtgcttttgttaatttaaaacaattaccatttttctattactctgacagtccatgtgagtctcatggaaaacaagtagtgtcagatatagattatgtaccactaaagtctgctacgtgtataacacgttgcaatttaggtggtgctgtctgtagacatcatgctaatgagtacagattgtatctcgatgcttataacatgatgatctcagctggctttagcttgtgggtttacaaacaatttgatacttataacctctggaacacttttacaagacttcagagtttagaaaatgtggcttttaatgttgtaaataagggacactttgatggacaacagggtgaagtaccagtttctatcattaataacactgtttacacaaaagttgatggtgttgatgtagaattgtttgaaaataaaacaacattacctgttaatgtagcatttgagctttgggctaagcgcaacattaaaccagtaccagaggtgaaaatactcaataatttgggtgtggacattgctgctaatactgtgatctgggactacaaaagagatgctccagcacatatatctactattggtgtttgttctatgactgacatagccaagaaaccaactgaaacgatttgtgcaccactcactgtcttttttgatggtagagttgatggtcaagtagacttatttagaaatgcccgtaatggtgttcttattacagaaggtagtgttaaaggtttacaaccatctgtaggtcccaaacaagctagtcttaatggagtcacattaattggagaagccgtaaaaacacagttcaattattataagaaagttgatggtgttgtccaacaattacctgaaacttactttactcagagtagaaatttacaagaatttaaacccaggagtcaaatggaaattgatttcttagaattagctatggatgaattcattgaacggtataaattagaaggctatgccttcgaacatatcgtttatggagattttagtcatagtcagttaggtggtttacatctactgattggactagctaaacgttttaaggaatcaccttttgaattagaagattttattcctatggacagtacagttaaaaactatttcataacagatgcgcaaacaggttcatctaagtgtgtgtgttctgttattgatttattacttgatgattttgttgaaataataaaatcccaagatttatctgtagtttctaaggttgtcaaagtgactattgactatacagaaatttcatttatgctttggtgtaaagatggccatgtagaaacattttacccaaaattacaatctagtcaagcgtggcaaccgggtgttgctatgcctaatctttacaaaatgcaaagaatgctattagaaaagtgtgaccttcaaaattatggtgatagtgcaacattacctaaaggcataatgatgaatgtcgcaaaatatactcaactgtgtcaatatttaaacacattaacattagctgtaccctataatatgagagttatacattttggtgctggttctgataaaggagttgcaccaggtacagctgttttaagacagtggttgcctacgggtacgctgcttgtcgattcagatcttaatgactttgtctctgatgcagattcaactttgattggtgattgtgcaactgtacatacagctaataaatgggatctcattattagtgatatgtacgaccctaagactaaaaatgttacaaaagaaaatgactctaaagagggttttttcacttacatttgtgggtttatacaacaaaagctagctcttggaggttccgtggctataaagataacagaacattcttggaatgctgatctttataagctcatgggacacttcgcatggtggacagcctttgttactaatgtgaatgcgtcatcatctgaagcatttttaattggatgtaattatcttggcaaaccacgcgaacaaatagatggttatgtcatgcatgcaaattacatattttggaggaatacaaatccaattcagttgtcttcctattctttatttgacatgagtaaatttccccttaaattaaggggtactgctgttatgtctttaaaagaaggtcaaatcaatgatatgattttatctcttcttagtaaaggtagacttataattagagaaaacaacagagttgttatttctagtgatgttcttgttaacaactaa

SEQ ID NO: 36 - RNA, 154 nt, artificial
  Artificial
ggcgccgucuuguugaccaacaguuuguugacuaaauaacgguuaacaagcuguuucagagaggacgcaaauaaaguccucuuuggaguaguuuguugauuuacuuuaaggagggcaaaaugggaagcuucgaucccgccgucguuuuacaacg

SEQ ID NO: 37 - RNA, 154 nt, artificial; identical to SEQ ID NO: 36
  Artificial

SEQ ID NO: 38 - RNA, 30 nt, severe acute respiratory syndrome coronavirus 2 isolate wuhan-hu-1 (sars-cov-2)
agucaacaaacuguuggucaacaagacggc

SEQ ID NO: 39 - DNA, 181 bp, artificial
  Artificial
tcataagctttaatacgactcactataggcgccgtcttgttgaccaacagtttgttgactaaataacggttaacaagctgtttcagagaggacgcaaataaagtcctctttggagtagtttgttgatttactttaaggagggcaaaatgggaagcttcgatcccgccgtcgttttacaacg

SEQ ID NO: 40 - DNA, 181 bp, artificial
  Artificial
tcataagctttaatacgactcactataggcgccgtcttgttgaccaacagtttgttgactaaataacggttaacaagctgtttcaaagaggacgcaaataaagtcctctttggagtagtttgttgatttactttaaggagggcaaaatgggaagcttcgatcccgccgtcgttttacaacg

SEQ ID NO: 41 - DNA, 3247 bp, artificial
  Artificial
tcataagctttaatacgactcactataggcgccgtcttgttgaccaacagtttgttgactaaataacggttaacaagctgtttcagagaggacgcaaataaagtcctctttggagtagtttgttgatttactttaaggagggcaaaatgggaagcttcgatcccgccgtcgttttacaacgtcgtgactgggaaaaccctggcgttacccaacttaatcgccttgcagcacatccccctttcgccagctggcgtaatagcgaagaggcccgcaccgatcgcccttcccaacagttgcgcagcctgaatggcgaatggcgctttgcctggtttccggcaccagaagcggtgccggaaagctggctggagtgcgatcttcctgaggccgatactgtcgtcgtcccctcaaactggcagatgcacggttacgatgcgcccatctacaccaacgtgacctatcccattacggtcaatccgccgtttgttcccacggagaatccgacgggttgttactcgctcacatttaatgttgatgaaagctggctacaggaaggccagacgcgaattatttttgatggcgttaactcggcgtttcatctgtggtgcaacgggcgctgggtcggttacggccaggacagtcgtttgccgtctgaatttgacctgagcgcatttttacgcgccggagaaaaccgcctcgcggtgatggtgctgcgctggagtgacggcagttatctggaagatcaggatatgtggcggatgagcggcattttccgtgacgtctcgttgctgcataaaccgactacacaaatcagcgatttccatgttgccactcgctttaatgatgatttcagccgcgctgtactggaggctgaagttcagatgtgcggcgagttgcgtgactacctacgggtaacagtttctttatggcagggtgaaacgcaggtcgccagcggcaccgcgcctttcggcggtgaaattatcgatgagcgtggtggttatgccgatcgcgtcacactacgtctgaacgtcgaaaacccgaaactgtggagcgccgaaatcccgaatctctatcgtgcggtggttgaactgcacaccgccgacggcacgctgattgaagcagaagcctgcgatgtcggtttccgcgaggtgcggattgaaaatggtctgctgctgctgaacggcaagccgttgctgattcgaggcgttaaccgtcacgagcatcatcctctgcatggtcaggtcatggatgagcagacgatggtgcaggatatcctgctgatgaagcagaacaactttaacgccgtgcgctgttcgcattatccgaaccatccgctgtggtacacgctgtgcgaccgctacggcctgtatgtggtggatgaagccaatattgaaacccacggcatggtgccaatgaatcgtctgaccgatgatccgcgctggctaccggcgatgagcgaacgcgtaacgcgaatggtgcagcgcgatcgtaatcacccgagtgtgatcatctggtcgctggggaatgaatcaggccacggcgctaatcacgacgcgctgtatcgctggatcaaatctgtcgatccttcccgcccggtgcagtatgaaggcggcggagccgacaccacggccaccgatattatttgcccgatgtacgcgcgcgtggatgaagaccagcccttcccggctgtgccgaaatggtccatcaaaaaatggctttcgctacctggagagacgcgcccgctgatcctttgcgaatacgcccacgcgatgggtaacagtcttggcggtttcgctaaatactggcaggcgtttcgtcagtatccccgtttacagggcggcttcgtctgggactgggtggatcagtcgctgattaaatatgatgaaaacggcaacccgtggtcggcttacggcggtgattttggcgatacgccgaacgatcgccagttctgtatgaacggtctggtctttgccgaccgcacgccgcatccagcgctgacggaagcaaaacaccagcagcagtttttccagttccgtttatccgggcaaaccatcgaagtgaccagcgaatacctgttccgtcatagcgataacgagctcctgcactggatggtggcgctggatggtaagccgctggcaagcggtgaagtgcctctggatgtcgctccacaaggtaaacagttgattgaactgcctgaactaccgcagccggagagcgccgggcaactctggctcacagtacgcgtagtgcaaccgaacgcgaccgcatggtcagaagccgggcacatcagcgcctggcagcagtggcgtctggcggaaaacctcagtgtgacgctccccgccgcgtcccacgccatcccgcatctgaccaccagcgaaatggatttttgcatcgagctgggtaataagcgttggcaatttaaccgccagtcaggctttctttcacagatgtggattggcgataaaaaacaactgctgacgccgctgcgcgatcagttcacccgtgcaccgctggataacgacattggcgtaagtgaagcgacccgcattgaccctaacgcctgggtcgaacgctggaaggcggcgggccattaccaggccgaagcagcgttgttgcagtgcacggcagatacacttgctgatgcggtgctgattacgaccgctcacgcgtggcagcatcaggggaaaaccttatttatcagccggaaaacctaccggattgatggtagtggtcaaatggcgattaccgttgatgttgaagtggcgagcgatacaccgcatccggcgcggattggcctgaactgccagctggcgcaggtagcagagcgggtaaactggctcggattagggccgcaagaaaactatcccgaccgccttactgccgcctgttttgaccgctgggatctgccattgtcagacatgtataccccgtacgtcttcccgagcgaaaacggtctgcgctgcgggacgcgcgaattgaattatggcccacaccagtggcgcggcgacttccagttcaacatcagccgctacagtcaacagcaactgatggaaaccagccatcgccatctgctgcacgcggaagaaggcacatggctgaatatcgacggtttccatatggggattggtggcgacgactcctggagcccgtcagtatcggcggaattccagctgagcgccggtcgctaccattaccagttggtctggtgtcaaaaataactagcataacccctctctaaacggaggggttt

SEQ ID NO: 42 - DNA, 3247 bp, artificial
  Artificial
tcataagctttaatacgactcactataggcgccgtcttgttgaccaacagtttgttgactaaataacggttaacaagctgtttcaaagaggacgcaaataaagtcctctttggagtagtttgttgatttactttaaggagggcaaaatgggaagcttcgatcccgccgtcgttttacaacgtcgtgactgggaaaaccctggcgttacccaacttaatcgccttgcagcacatccccctttcgccagctggcgtaatagcgaagaggcccgcaccgatcgcccttcccaacagttgcgcagcctgaatggcgaatggcgctttgcctggtttccggcaccagaagcggtgccggaaagctggctggagtgcgatcttcctgaggccgatactgtcgtcgtcccctcaaactggcagatgcacggttacgatgcgcccatctacaccaacgtgacctatcccattacggtcaatccgccgtttgttcccacggagaatccgacgggttgttactcgctcacatttaatgttgatgaaagctggctacaggaaggccagacgcgaattatttttgatggcgttaactcggcgtttcatctgtggtgcaacgggcgctgggtcggttacggccaggacagtcgtttgccgtctgaatttgacctgagcgcatttttacgcgccggagaaaaccgcctcgcggtgatggtgctgcgctggagtgacggcagttatctggaagatcaggatatgtggcggatgagcggcattttccgtgacgtctcgttgctgcataaaccgactacacaaatcagcgatttccatgttgccactcgctttaatgatgatttcagccgcgctgtactggaggctgaagttcagatgtgcggcgagttgcgtgactacctacgggtaacagtttctttatggcagggtgaaacgcaggtcgccagcggcaccgcgcctttcggcggtgaaattatcgatgagcgtggtggttatgccgatcgcgtcacactacgtctgaacgtcgaaaacccgaaactgtggagcgccgaaatcccgaatctctatcgtgcggtggttgaactgcacaccgccgacggcacgctgattgaagcagaagcctgcgatgtcggtttccgcgaggtgcggattgaaaatggtctgctgctgctgaacggcaagccgttgctgattcgaggcgttaaccgtcacgagcatcatcctctgcatggtcaggtcatggatgagcagacgatggtgcaggatatcctgctgatgaagcagaacaactttaacgccgtgcgctgttcgcattatccgaaccatccgctgtggtacacgctgtgcgaccgctacggcctgtatgtggtggatgaagccaatattgaaacccacggcatggtgccaatgaatcgtctgaccgatgatccgcgctggctaccggcgatgagcgaacgcgtaacgcgaatggtgcagcgcgatcgtaatcacccgagtgtgatcatctggtcgctggggaatgaatcaggccacggcgctaatcacgacgcgctgtatcgctggatcaaatctgtcgatccttcccgcccggtgcagtatgaaggcggcggagccgacaccacggccaccgatattatttgcccgatgtacgcgcgcgtggatgaagaccagcccttcccggctgtgccgaaatggtccatcaaaaaatggctttcgctacctggagagacgcgcccgctgatcctttgcgaatacgcccacgcgatgggtaacagtcttggcggtttcgctaaatactggcaggcgtttcgtcagtatccccgtttacagggcggcttcgtctgggactgggtggatcagtcgctgattaaatatgatgaaaacggcaacccgtggtcggcttacggcggtgattttggcgatacgccgaacgatcgccagttctgtatgaacggtctggtctttgccgaccgcacgccgcatccagcgctgacggaagcaaaacaccagcagcagtttttccagttccgtttatccgggcaaaccatcgaagtgaccagcgaatacctgttccgtcatagcgataacgagctcctgcactggatggtggcgctggatggtaagccgctggcaagcggtgaagtgcctctggatgtcgctccacaaggtaaacagttgattgaactgcctgaactaccgcagccggagagcgccgggcaactctggctcacagtacgcgtagtgcaaccgaacgcgaccgcatggtcagaagccgggcacatcagcgcctggcagcagtggcgtctggcggaaaacctcagtgtgacgctccccgccgcgtcccacgccatcccgcatctgaccaccagcgaaatggatttttgcatcgagctgggtaataagcgttggcaatttaaccgccagtcaggctttctttcacagatgtggattggcgataaaaaacaactgctgacgccgctgcgcgatcagttcacccgtgcaccgctggataacgacattggcgtaagtgaagcgacccgcattgaccctaacgcctgggtcgaacgctggaaggcggcgggccattaccaggccgaagcagcgttgttgcagtgcacggcagatacacttgctgatgcggtgctgattacgaccgctcacgcgtggcagcatcaggggaaaaccttatttatcagccggaaaacctaccggattgatggtagtggtcaaatggcgattaccgttgatgttgaagtggcgagcgatacaccgcatccggcgcggattggcctgaactgccagctggcgcaggtagcagagcgggtaaactggctcggattagggccgcaagaaaactatcccgaccgccttactgccgcctgttttgaccgctgggatctgccattgtcagacatgtataccccgtacgtcttcccgagcgaaaacggtctgcgctgcgggacgcgcgaattgaattatggcccacaccagtggcgcggcgacttccagttcaacatcagccgctacagtcaacagcaactgatggaaaccagccatcgccatctgctgcacgcggaagaaggcacatggctgaatatcgacggtttccatatggggattggtggcgacgactcctggagcccgtcagtatcggcggaattccagctgagcgccggtcgctaccattaccagttggtctggtgtcaaaaataactagcataacccctctctaaacggaggggttt

SEQ ID NO: 43 - DNA, 366 bp, severe acute respiratory syndrome coronavirus 2 isolate wuhan-hu-1 (sars-cov-2)
atgaaatttcttgttttcttaggaatcatcacaactgtagctgcatttcaccaagaatgtagtttacagtcatgtactcaacatcaaccatatgtagttgatgacccgtgtcctattcacttctattctaaatggtatattagagtaggagctagaaaatcagcacctttaattgaattgtgcgtggatgaggctggttctaaatcacccattcagtacatcgatatcggtaattatacagtttcctgtttaccttttacaattaattgccaggaacctaaattgggtagtcttgtagtgcgttgttcgttctatgaagactttttagagtatcatgacgttcgtgttgttttagatttcatctaa

SEQ ID NO: 44 - RNA, 154 nt, artificial
  Artificial
ggcgguuaauggguuguugguuagcgaggcggcauaaaucgccgucuugcuggccuagggaggcggccagguacaucgccuccuuagguugguaagacgguaacuuaaggaggcgaaaaugcagaaccuggcggcagcgcaaaagaugcguaaa

SEQ ID NO: 45 - RNA, 153 nt, artificial
  Artificial
ggcccuauucacuuuauucuaaaugguauauuuaagacugguauaccguuuagauaaggagggcaccgggguauuguccuccuuguuuggacgguauauccgaauaaggaggacaagaugcaaaaccuggcggcagcgcaaaagaugcguaaa

SEQ ID NO: 46 - RNA, 30 nt, severe acute respiratory syndrome coronavirus 2 isolate wuhan-hu-1 (sars-cov-2)
gccgucuuguugaccaacaguuuguugacu

SEQ ID NO: 47 - RNA, 30 nt, severe acute respiratory syndrome coronavirus 2 isolate wuhan-hu-1 (sars-cov-2)
aauauaccauuuagaauagaagugaauagg

SEQ ID NO: 48 - DNA, 181 bp, artificial
  Artificial
tcataagctttaatacgactcactataggcggttaatgggttgttggttagcgaggcggcataaatcgccgtcttgctggcctagggaggcggccaggtacatcgcctccttaggttggtaagacggtaacttaaggaggcgaaaatgcagaacctggcggcagcgcaaaagatgcgtaaa

SEQ ID NO: 49 - DNA, 181 bp, artificial
  Artificial
tcataagctttaatacgactcactataggccctattcacttctattctaaatggtatatttaagactggtataccgtttagataaggagggcaccggggtattgtcctccttgtttggacggtatatccgaataaggaggacaagatgcaaaacctggcggcagcgcaaaagatgcgtaaa

SEQ ID NO: 50 - DNA, 1057 bp, artificial
  Artificial
tcataagctttaatacgactcactataggcggttaatgggttgttggttagcgaggcggcataaatcgccgtcttgctggcctagggaggcggccaggtacatcgcctccttaggttggtaagacggtaacttaaggaggcgaaaatgcagaacctggcggcagcgcaaaagatgcgtaaaggagaagaacttttcactggagttgtcccaattcttgttgaattagatggtgatgttaatgggcacaaattttctgtcagtggagagggtgaaggtgatgcaacatacggaaaacttacccttaaatttatttgcactactggaaaactacctgttccgtggccaacacttgtcactactttcggttatggtgttcaatgctttgcgagatacccagatcacatgaaacagcatgactttttcaagagtgccatgcccgaaggttacgtacaggaaagaactatatttttcaaagatgacgggaactacaagacacgtgctgaagtcaagtttgaaggtgatacccttgttaatagaatcgagttaaaaggtattgattttaaagaagatggaaacattcttggacacaaattggaatacaactataactcacacaatgtatacatcatggcagacaaacaaaagaatggaatcaaagttaacttcaaaattagacacaacattgaagatggaagcgttcaactagcagaccattatcaacaaaatactccgattggcgatggccctgtccttttaccagacaaccattacctgtccacacaatctgccctttcgaaagatcccaacgaaaagagagaccacatggtccttcttgagtttgtaaccgctgctgggattacacatggcatggatgaactatacaaaaggcctgcagcaaacgacgaaaactacgctgcatcagtttaataataagataaaccagagcggcacggcaagcagagtatacgagattcggtagccaccgctgagcaataactagcataaccccttggggcctctaaacgggtcttgaggggttttttgcatatgcaacgg

SEQ ID NO: 51 - DNA, 1057 bp, artificial
  Artificial
tcataagctttaatacgactcactataggcagttaagttatttatggctgagagtggactgtaaataagtccgctctcagtcgaaggaggcgtcttttgcaaacgcctcctttggttgagagcggattgactaaaggaggcgtatatgtcgaacctggcggcagcgcaaaagatgcgtaaaggagaagaacttttcactggagttgtcccaattcttgttgaattagatggtgatgttaatgggcacaaattttctgtcagtggagagggtgaaggtgatgcaacatacggaaaacttacccttaaatttatttgcactactggaaaactacctgttccgtggccaacacttgtcactactttcggttatggtgttcaatgctttgcgagatacccagatcacatgaaacagcatgactttttcaagagtgccatgcccgaaggttacgtacaggaaagaactatatttttcaaagatgacgggaactacaagacacgtgctgaagtcaagtttgaaggtgatacccttgttaatagaatcgagttaaaaggtattgattttaaagaagatggaaacattcttggacacaaattggaatacaactataactcacacaatgtatacatcatggcagacaaacaaaagaatggaatcaaagttaacttcaaaattagacacaacattgaagatggaagcgttcaactagcagaccattatcaacaaaatactccgattggcgatggccctgtccttttaccagacaaccattacctgtccacacaatctgccctttcgaaagatcccaacgaaaagagagaccacatggtccttcttgagtttgtaaccgctgctgggattacacatggcatggatgaactatacaaaaggcctgcagcaaacgacgaaaactacgctgcatcagtttaataataagataaaccagagcggcacggcaagcagagtatacgagattcggtagccaccgctgagcaataactagcataaccccttggggcctctaaacgggtcttgaggggttttttgcatatgcaacgg

SEQ ID NO: 52 - DNA, 444 bp, Artificial Sequence
  Artificial
atggcaaacctggacaagatgctgaataccacagtaacagaggtgcggcagttcctgcaggtggacagagtgtgcgtgttccagtttgaggaggattatagcggagtggtggtggtggaggccgtggacgataggtggatctccatcctgaagacccaggtgcgggatagatacttcatggagacaaggggcgaggagtattctcacggccgctaccaggccatcgccgacatctacaccgcaaacctgacagagtgctacagggatctgctgacacagtttcaggtgagagcaatcctggccgtgcccatcctgcagggcaagaagctgtggggcctgttggtggcacaccagctggcggcccctagacagtggcagacctgggagatcgactttctgaagcagcaggccgtggtggtgggcatcgccatccagcagagctaa

SEQ ID NO: 53 - RNA, 595 nt, Artificial Sequence
  Artificial
ggcgguugauggguuguuggucaacagggcggcgauaaucgccguucuguuggcuagcaaggaggaaaauauggcaaaccuggacaagaugcugaauaccacaguaacagaggugcggcaguuccugcagguggacagagugugcguguuccaguuugaggaggauuauagcggagugguggugguggaggccguggacgauagguggaucuccauccugaagacccaggugcgggauagauacuucauggagacaaggggcgaggaguauucucacggccgcuaccaggccaucgccgacaucuacaccgcaaaccugacagagugcuacagggaucugcugacacaguuucaggugagagcaauccuggccgugcccauccugcagggcaagaagcuguggggccuguugguggcacaccagcuggcggccccuagacaguggcagaccugggagaucgacuuucugaagcagcaggccgugguggugggcaucgccauccagcagagcuaauuuccuccuuguuagccaauagaauggucuaacaaggaggaaacaauguauacaacaaaccuggcggcagcgcaaaagaug

SEQ ID NO: 54 - RNA, 595 nt, Artificial Sequence
  Artificial
ggcgguugauggguuguuggucaacagggcggcgauaauugccguucuguuggcuagcaaggaggaaaauauggcaaaccuggacaagaugcugaauaccacaguaacagaggugcggcaguuccugcagguggacagagugugcguguuccaguuugaggaggauuauagcggagugguggugguggaggccguggacgauagguggaucuccauccugaagacccaggugcgggauagauacuucauggagacaaggggcgaggaguauucucacggccgcuaccaggccaucgccgacaucuacaccgcaaaccugacagagugcuacagggaucugcugacacaguuucaggugagagcaauccuggccgugcccauccugcagggcaagaagcuguggggccuguugguggcacaccagcuggcggccccuagacaguggcagaccugggagaucgacuuucugaagcagcaggccgugguggugggcaucgccauccagcagagcuaauuuccuccuuguuagccaauagaauggucuaacaaggaggaaacaauguauacaacaaaccuggcggcagcgcaaaagaug

SEQ ID NO: 55 - DNA, 115 bp, Artificial Sequence
  Artificial
tcataagctttaatacgactcactataggcggttgatgggttgttggtcaacagggcggcgataatcgccgttctgttggctagcaaggaggaaaatatggcaaacctggacaag

SEQ ID NO: 56 - DNA, 115 bp, Artificial Sequence
  Artificial
tcataagctttaatacgactcactataggcggttgatgggttgttggtcaacagggcggcgataattgccgttctgttggctagcaaggaggaaaatatggcaaacctggacaag

SEQ ID NO: 57 - DNA, 52 bp, Artificial Sequence
  Artificial
cagctggtgtgccaccaacaggccccacagcttcttgccctgcaggatgggc

SEQ ID NO: 58 - DNA, 454 bp, Artificial Sequence
  Artificial
tcataagctttaatacgactcactataggcggttgatgggttgttggtcaacagggcggcgataatcgccgttctgttggctagcaaggaggaaaatatggcaaacctggacaagatgctgaataccacagtaacagaggtgcggcagttcctgcaggtggacagagtgtgcgtgttccagtttgaggaggattatagcggagtggtggtggtggaggccgtggacgataggtggatctccatcctgaagacccaggtgcgggatagatacttcatggagacaaggggcgaggagtattctcacggccgctaccaggccatcgccgacatctacaccgcaaacctgacagagtgctacagggatctgctgacacagtttcaggtgagagcaatcctggccgtgcccatcctgcagggcaagaagctgtggggcctgttggtggcacaccagctg

SEQ ID NO: 59 - DNA, 454 bp, Artificial Sequence
  Artificial
tcataagctttaatacgactcactataggcggttgatgggttgttggtcaacagggcggcgataattgccgttctgttggctagcaaggaggaaaatatggcaaacctggacaagatgctgaataccacagtaacagaggtgcggcagttcctgcaggtggacagagtgtgcgtgttccagtttgaggaggattatagcggagtggtggtggtggaggccgtggacgataggtggatctccatcctgaagacccaggtgcgggatagatacttcatggagacaaggggcgaggagtattctcacggccgctaccaggccatcgccgacatctacaccgcaaacctgacagagtgctacagggatctgctgacacagtttcaggtgagagcaatcctggccgtgcccatcctgcagggcaagaagctgtggggcctgttggtggcacaccagctg

SEQ ID NO: 60 - DNA, 200 bp, Artificial Sequence
  Artificial
agctgtggggcctgttggtggcacaccagctggcggcccctagacagtggcagacctgggagatcgactttctgaagcagcaggccgtggtggtgggcatcgccatccagcagagctaatttcctccttgttagccaatagaatggtctaacaaggaggaaacaatgtatacaacaaacctggcggcagcgcaaaagatg

SEQ ID NO: 61 - DNA, 1082 bp, Artificial Sequence
  Artificial
agctgtggggcctgttggtggcacaccagctggcggcccctagacagtggcagacctgggagatcgactttctgaagcagcaggccgtggtggtgggcatcgccatccagcagagctaatttcctccttgttagccaatagaatggtctaacaaggaggaaacaatgtatacaacaaacctggcggcagcgcaaaagatgcgtaaaggagaagaacttttcactggagttgtcccaattcttgttgaattagatggtgatgttaatgggcacaaattttctgtcagtggagagggtgaaggtgatgcaacatacggaaaacttacccttaaatttatttgcactactggaaaactacctgttccgtggccaacacttgtcactactttcggttatggtgttcaatgctttgcgagatacccagatcacatgaaacagcatgactttttcaagagtgccatgcccgaaggttacgtacaggaaagaactatatttttcaaagatgacgggaactacaagacacgtgctgaagtcaagtttgaaggtgatacccttgttaatagaatcgagttaaaaggtattgattttaaagaagatggaaacattcttggacacaaattggaatacaactataactcacacaatgtatacatcatggcagacaaacaaaagaatggaatcaaagttaacttcaaaattagacacaacattgaagatggaagcgttcaactagcagaccattatcaacaaaatactccgattggcgatggccctgtccttttaccagacaaccattacctgtccacacaatctgccctttcgaaagatcccaacgaaaagagagaccacatggtccttcttgagtttgtaaccgctgctgggattacacatggcatggatgaactatacaaaaggcctgcagcaaacgacgaaaactacgctgcatcagtttaataataagataaaccagagcggcacggcaagcagagtatacgagattcggtagccaccgctgagcaataactagcataaccccttggggcctctaaacgggtcttgaggggttttttgcatatgcaacgg

SEQ ID NO: 62 - DNA, 1082 bp, Artificial Sequence; identical to SEQ ID NO: 61
  Artificial

SEQ ID NO: 63 - DNA, 21 bp, Artificial Sequence
  Artificial
tcataagctttaatacgactc

SEQ ID NO: 64 - DNA, 21 bp, Artificial Sequence
  Artificial
ccgttgcatatgcaaaaaacc

SEQ ID NO: 65 - DNA, 1504 bp, Artificial Sequence
  Artificial
tcataagctttaatacgactcactataggcggttgatgggttgttggtcaacagggcggcgataatcgccgttctgttggctagcaaggaggaaaatatggcaaacctggacaagatgctgaataccacagtaacagaggtgcggcagttcctgcaggtggacagagtgtgcgtgttccagtttgaggaggattatagcggagtggtggtggtggaggccgtggacgataggtggatctccatcctgaagacccaggtgcgggatagatacttcatggagacaaggggcgaggagtattctcacggccgctaccaggccatcgccgacatctacaccgcaaacctgacagagtgctacagggatctgctgacacagtttcaggtgagagcaatcctggccgtgcccatcctgcagggcaagaagctgtggggcctgttggtggcacaccagctggcggcccctagacagtggcagacctgggagatcgactttctgaagcagcaggccgtggtggtgggcatcgccatccagcagagctaatttcctccttgttagccaatagaatggtctaacaaggaggaaacaatgtatacaacaaacctggcggcagcgcaaaagatgcgtaaaggagaagaacttttcactggagttgtcccaattcttgttgaattagatggtgatgttaatgggcacaaattttctgtcagtggagagggtgaaggtgatgcaacatacggaaaacttacccttaaatttatttgcactactggaaaactacctgttccgtggccaacacttgtcactactttcggttatggtgttcaatgctttgcgagatacccagatcacatgaaacagcatgactttttcaagagtgccatgcccgaaggttacgtacaggaaagaactatatttttcaaagatgacgggaactacaagacacgtgctgaagtcaagtttgaaggtgatacccttgttaatagaatcgagttaaaaggtattgattttaaagaagatggaaacattcttggacacaaattggaatacaactataactcacacaatgtatacatcatggcagacaaacaaaagaatggaatcaaagttaacttcaaaattagacacaacattgaagatggaagcgttcaactagcagaccattatcaacaaaatactccgattggcgatggccctgtccttttaccagacaaccattacctgtccacacaatctgccctttcgaaagatcccaacgaaaagagagaccacatggtccttcttgagtttgtaaccgctgctgggattacacatggcatggatgaactatacaaaaggcctgcagcaaacgacgaaaactacgctgcatcagtttaataataagataaaccagagcggcacggcaagcagagtatacgagattcggtagccaccgctgagcaataactagcataaccccttggggcctctaaacgggtcttgaggggttttttgcatatgcaacgg

SEQ ID NO: 66 - DNA, 1504 bp, Artificial Sequence
  Artificial
tcataagctttaatacgactcactataggcggttgatgggttgttggtcaacagggcggcgataattgccgttctgttggctagcaaggaggaaaatatggcaaacctggacaagatgctgaataccacagtaacagaggtgcggcagttcctgcaggtggacagagtgtgcgtgttccagtttgaggaggattatagcggagtggtggtggtggaggccgtggacgataggtggatctccatcctgaagacccaggtgcgggatagatacttcatggagacaaggggcgaggagtattctcacggccgctaccaggccatcgccgacatctacaccgcaaacctgacagagtgctacagggatctgctgacacagtttcaggtgagagcaatcctggccgtgcccatcctgcagggcaagaagctgtggggcctgttggtggcacaccagctggcggcccctagacagtggcagacctgggagatcgactttctgaagcagcaggccgtggtggtgggcatcgccatccagcagagctaatttcctccttgttagccaatagaatggtctaacaaggaggaaacaatgtatacaacaaacctggcggcagcgcaaaagatgcgtaaaggagaagaacttttcactggagttgtcccaattcttgttgaattagatggtgatgttaatgggcacaaattttctgtcagtggagagggtgaaggtgatgcaacatacggaaaacttacccttaaatttatttgcactactggaaaactacctgttccgtggccaacacttgtcactactttcggttatggtgttcaatgctttgcgagatacccagatcacatgaaacagcatgactttttcaagagtgccatgcccgaaggttacgtacaggaaagaactatatttttcaaagatgacgggaactacaagacacgtgctgaagtcaagtttgaaggtgatacccttgttaatagaatcgagttaaaaggtattgattttaaagaagatggaaacattcttggacacaaattggaatacaactataactcacacaatgtatacatcatggcagacaaacaaaagaatggaatcaaagttaacttcaaaattagacacaacattgaagatggaagcgttcaactagcagaccattatcaacaaaatactccgattggcgatggccctgtccttttaccagacaaccattacctgtccacacaatctgccctttcgaaagatcccaacgaaaagagagaccacatggtccttcttgagtttgtaaccgctgctgggattacacatggcatggatgaactatacaaaaggcctgcagcaaacgacgaaaactacgctgcatcagtttaataataagataaaccagagcggcacggcaagcagagtatacgagattcggtagccaccgctgagcaataactagcataaccccttggggcctctaaacgggtcttgaggggttttttgcatatgcaacgg

SEQ ID NO: 67 - RNA, 595 nt, Artificial Sequence
ggcaaguuugauguggcugugcugcguguauggggauaacuuguauguguggcgcagcaaggaggaaaauauggcaaaccuggacaagaugcugaauaccacaguaacagaggugcggcaguuccugcagguggacagagugugcguguuccaguuugaggaggauuauagcggagugguggugguggaggccguggacgauagguggaucuccauccugaagacccaggugcgggauagauacuucauggagacaaggggcgaggaguauucucacggccgcuaccaggccaucgccgacaucuacaccgcaaaccugacagagugcuacagggaucugcugacacaguuucaggugagagcaauccuggccgugcccauccugcagggcaagaagcuguggggccuguugguggcacaccagcuggcggccccuagacaguggcagaccugggagaucgacuuucugaagcagcaggccgugguggugggcaucgccauccagcagagcuaauuuccuccuuguugcgcuguauguacgggcaauaaggaggaaauaaugucaaccaccaaccuggcggcagcgcaaaagaug

SEQ ID NO: 68 - RNA, 595 nt, Artificial Sequence
ggcuaguuguguuguguguaugaagaaggccuugaauaacggggucuucuuugugguuaaggaggaaaauauggcaaaccuggacaagaugcugaauaccacaguaacagaggugcggcaguuccugcagguggacagagugugcguguuccaguuugaggaggauuauagcggagugguggugguggaggccguggacgauagguggaucuccauccugaagacccaggugcgggauagauacuucauggagacaaggggcgaggaguauucucacggccgcuaccaggccaucgccgacaucuacaccgcaaaccugacagagugcuacagggaucugcugacacaguuucaggugagagcaauccuggccgugcccauccugcagggcaagaagcuguggggccuguugguggcacaccagcuggcggccccuagacaguggcagaccugggagaucgacuuucugaagcagcaggccgugguggugggcaucgccauccagcagagcuaauuuccuccuuagucacgaagaagacuucugacuaaggagggaauaaugucgaagacgaaccuggcggcagcgcaaaagaug

SEQ ID NO: 69 - RNA, 595 nt, Artificial Sequence
ggcuaguuguguuguguguaugaagaaggccuugaauaacggggucuucuucgugguuaaggaggaaaauauggcaaaccuggacaagaugcugaauaccacaguaacagaggugcggcaguuccugcagguggacagagugugcguguuccaguuugaggaggauuauagcggagugguggugguggaggccguggacgauagguggaucuccauccugaagacccaggugcgggauagauacuucauggagacaaggggcgaggaguauucucacggccgcuaccaggccaucgccgacaucuacaccgcaaaccugacagagugcuacagggaucugcugacacaguuucaggugagagcaauccuggccgugcccauccugcagggcaagaagcuguggggccuguugguggcacaccagcuggcggccccuagacaguggcagaccugggagaucgacuuucugaagcagcaggccgugguggugggcaucgccauccagcagagcuaauuuccuccuuagucacgaagaagacuucugacuaaggagggaauaaugucgaagacgaaccuggcggcagcgcaaaagaug

SEQ ID NO: 70 - RNA, 595 nt, Artificial Sequence
ggcuaguuguguuguguguaugaagagggccuugaauaacggggucuucuucgugguuaaggaggaaaauauggcaaaccuggacaagaugcugaauaccacaguaacagaggugcggcaguuccugcagguggacagagugugcguguuccaguuugaggaggauuauagcggagugguggugguggaggccguggacgauagguggaucuccauccugaagacccaggugcgggauagauacuucauggagacaaggggcgaggaguauucucacggccgcuaccaggccaucgccgacaucuacaccgcaaaccugacagagugcuacagggaucugcugacacaguuucaggugagagcaauccuggccgugcccauccugcagggcaagaagcuguggggccuguugguggcacaccagcuggcggccccuagacaguggcagaccugggagaucgacuuucugaagcagcaggccgugguggugggcaucgccauccagcagagcuaauuuccuccuuagucacgaagaagacuucugacuaaggagggaauaaugucgaagacgaaccuggcggcagcgcaaaagaug

SEQ ID NO: 71 - DNA, 115 bp, Artificial Sequence
tcataagctttaatacgactcactataggcaagtttgatgtggctgtgctgcgtgtatggggataacttgtatgtgtggcgcagcaaggaggaaaatatggcaaacctggacaag

SEQ ID NO: 72 - DNA, 115 bp, Artificial Sequence
tcataagctttaatacgactcactataggctagttgtgttgtgtgtatgaagaaggccttgaataacggggtcttctttgtggttaaggaggaaaatatggcaaacctggacaag

SEQ ID NO: 73 - DNA, 115 bp, Artificial Sequence
tcataagctttaatacgactcactataggctagttgtgttgtgtgtatgaagaaggccttgaataacggggtcttcttcgtggttaaggaggaaaatatggcaaacctggacaag

SEQ ID NO: 74 - DNA, 115 bp, Artificial Sequence
tcataagctttaatacgactcactataggctagttgtgttgtgtgtatgaagagggccttgaataacggggtcttcttcgtggttaaggaggaaaatatggcaaacctggacaag

SEQ ID NO: 75 - DNA, 454 bp, Artificial Sequence
tcataagctttaatacgactcactataggcaagtttgatgtggctgtgctgcgtgtatggggataacttgtatgtgtggcgcagcaaggaggaaaatatggcaaacctggacaagatgctgaataccacagtaacagaggtgcggcagttcctgcaggtggacagagtgtgcgtgttccagtttgaggaggattatagcggagtggtggtggtggaggccgtggacgataggtggatctccatcctgaagacccaggtgcgggatagatacttcatggagacaaggggcgaggagtattctcacggccgctaccaggccatcgccgacatctacaccgcaaacctgacagagtgctacagggatctgctgacacagtttcaggtgagagcaatcctggccgtgcccatcctgcagggcaagaagctgtggggcctgttggtggcacaccagctg

SEQ ID NO: 76 - DNA, 454 bp, Artificial Sequence
tcataagctttaatacgactcactataggctagttgtgttgtgtgtatgaagaaggccttgaataacggggtcttctttgtggttaaggaggaaaatatggcaaacctggacaagatgctgaataccacagtaacagaggtgcggcagttcctgcaggtggacagagtgtgcgtgttccagtttgaggaggattatagcggagtggtggtggtggaggccgtggacgataggtggatctccatcctgaagacccaggtgcgggatagatacttcatggagacaaggggcgaggagtattctcacggccgctaccaggccatcgccgacatctacaccgcaaacctgacagagtgctacagggatctgctgacacagtttcaggtgagagcaatcctggccgtgcccatcctgcagggcaagaagctgtggggcctgttggtggcacaccagctg

SEQ ID NO: 77 - DNA, 454 bp, Artificial Sequence
tcataagctttaatacgactcactataggctagttgtgttgtgtgtatgaagaaggccttgaataacggggtcttcttcgtggttaaggaggaaaatatggcaaacctggacaagatgctgaataccacagtaacagaggtgcggcagttcctgcaggtggacagagtgtgcgtgttccagtttgaggaggattatagcggagtggtggtggtggaggccgtggacgataggtggatctccatcctgaagacccaggtgcgggatagatacttcatggagacaaggggcgaggagtattctcacggccgctaccaggccatcgccgacatctacaccgcaaacctgacagagtgctacagggatctgctgacacagtttcaggtgagagcaatcctggccgtgcccatcctgcagggcaagaagctgtggggcctgttggtggcacaccagctg

SEQ ID NO: 78 - DNA, 454 bp, Artificial Sequence
tcataagctttaatacgactcactataggctagttgtgttgtgtgtatgaagagggccttgaataacggggtcttcttcgtggttaaggaggaaaatatggcaaacctggacaagatgctgaataccacagtaacagaggtgcggcagttcctgcaggtggacagagtgtgcgtgttccagtttgaggaggattatagcggagtggtggtggtggaggccgtggacgataggtggatctccatcctgaagacccaggtgcgggatagatacttcatggagacaaggggcgaggagtattctcacggccgctaccaggccatcgccgacatctacaccgcaaacctgacagagtgctacagggatctgctgacacagtttcaggtgagagcaatcctggccgtgcccatcctgcagggcaagaagctgtggggcctgttggtggcacaccagctg

SEQ ID NO: 79 - DNA, 200 bp, Artificial Sequence
agctgtggggcctgttggtggcacaccagctggcggcccctagacagtggcagacctgggagatcgactttctgaagcagcaggccgtggtggtgggcatcgccatccagcagagctaatttcctccttgttgcgctgtatgtacgggcaataaggaggaaataatgtcaaccaccaacctggcggcagcgcaaaagatg

SEQ ID NO: 80 - DNA, 200 bp, Artificial Sequence
agctgtggggcctgttggtggcacaccagctggcggcccctagacagtggcagacctgggagatcgactttctgaagcagcaggccgtggtggtgggcatcgccatccagcagagctaatttcctccttagtcacgaagaagacttctgactaaggagggaataatgtcgaagacgaacctggcggcagcgcaaaagatg

SEQ ID NO: 81 - DNA, 1082 bp, Artificial Sequence
agctgtggggcctgttggtggcacaccagctggcggcccctagacagtggcagacctgggagatcgactttctgaagcagcaggccgtggtggtgggcatcgccatccagcagagctaatttcctccttgttgcgctgtatgtacgggcaataaggaggaaataatgtcaaccaccaacctggcggcagcgcaaaagatgcgtaaaggagaagaacttttcactggagttgtcccaattcttgttgaattagatggtgatgttaatgggcacaaattttctgtcagtggagagggtgaaggtgatgcaacatacggaaaacttacccttaaatttatttgcactactggaaaactacctgttccgtggccaacacttgtcactactttcggttatggtgttcaatgctttgcgagatacccagatcacatgaaacagcatgactttttcaagagtgccatgcccgaaggttacgtacaggaaagaactatatttttcaaagatgacgggaactacaagacacgtgctgaagtcaagtttgaaggtgatacccttgttaatagaatcgagttaaaaggtattgattttaaagaagatggaaacattcttggacacaaattggaatacaactataactcacacaatgtatacatcatggcagacaaacaaaagaatggaatcaaagttaacttcaaaattagacacaacattgaagatggaagcgttcaactagcagaccattatcaacaaaatactccgattggcgatggccctgtccttttaccagacaaccattacctgtccacacaatctgccctttcgaaagatcccaacgaaaagagagaccacatggtccttcttgagtttgtaaccgctgctgggattacacatggcatggatgaactatacaaaaggcctgcagcaaacgacgaaaactacgctgcatcagtttaataataagataaaccagagcggcacggcaagcagagtatacgagattcggtagccaccgctgagcaataactagcataaccccttggggcctctaaacgggtcttgaggggttttttgcatatgcaacgg

SEQ ID NO: 82 - DNA, 1082 bp, Artificial Sequence
agctgtggggcctgttggtggcacaccagctggcggcccctagacagtggcagacctgggagatcgactttctgaagcagcaggccgtggtggtgggcatcgccatccagcagagctaatttcctccttagtcacgaagaagacttctgactaaggagggaataatgtcgaagacgaacctggcggcagcgcaaaagatgcgtaaaggagaagaacttttcactggagttgtcccaattcttgttgaattagatggtgatgttaatgggcacaaattttctgtcagtggagagggtgaaggtgatgcaacatacggaaaacttacccttaaatttatttgcactactggaaaactacctgttccgtggccaacacttgtcactactttcggttatggtgttcaatgctttgcgagatacccagatcacatgaaacagcatgactttttcaagagtgccatgcccgaaggttacgtacaggaaagaactatatttttcaaagatgacgggaactacaagacacgtgctgaagtcaagtttgaaggtgatacccttgttaatagaatcgagttaaaaggtattgattttaaagaagatggaaacattcttggacacaaattggaatacaactataactcacacaatgtatacatcatggcagacaaacaaaagaatggaatcaaagttaacttcaaaattagacacaacattgaagatggaagcgttcaactagcagaccattatcaacaaaatactccgattggcgatggccctgtccttttaccagacaaccattacctgtccacacaatctgccctttcgaaagatcccaacgaaaagagagaccacatggtccttcttgagtttgtaaccgctgctgggattacacatggcatggatgaactatacaaaaggcctgcagcaaacgacgaaaactacgctgcatcagtttaataataagataaaccagagcggcacggcaagcagagtatacgagattcggtagccaccgctgagcaataactagcataaccccttggggcctctaaacgggtcttgaggggttttttgcatatgcaacgg

SEQ ID NO: 83 - DNA, 1504 bp, Artificial Sequence
tcataagctttaatacgactcactataggcaagtttgatgtggctgtgctgcgtgtatggggataacttgtatgtgtggcgcagcaaggaggaaaatatggcaaacctggacaagatgctgaataccacagtaacagaggtgcggcagttcctgcaggtggacagagtgtgcgtgttccagtttgaggaggattatagcggagtggtggtggtggaggccgtggacgataggtggatctccatcctgaagacccaggtgcgggatagatacttcatggagacaaggggcgaggagtattctcacggccgctaccaggccatcgccgacatctacaccgcaaacctgacagagtgctacagggatctgctgacacagtttcaggtgagagcaatcctggccgtgcccatcctgcagggcaagaagctgtggggcctgttggtggcacaccagctggcggcccctagacagtggcagacctgggagatcgactttctgaagcagcaggccgtggtggtgggcatcgccatccagcagagctaatttcctccttgttgcgctgtatgtacgggcaataaggaggaaataatgtcaaccaccaacctggcggcagcgcaaaagatgcgtaaaggagaagaacttttcactggagttgtcccaattcttgttgaattagatggtgatgttaatgggcacaaattttctgtcagtggagagggtgaaggtgatgcaacatacggaaaacttacccttaaatttatttgcactactggaaaactacctgttccgtggccaacacttgtcactactttcggttatggtgttcaatgctttgcgagatacccagatcacatgaaacagcatgactttttcaagagtgccatgcccgaaggttacgtacaggaaagaactatatttttcaaagatgacgggaactacaagacacgtgctgaagtcaagtttgaaggtgatacccttgttaatagaatcgagttaaaaggtattgattttaaagaagatggaaacattcttggacacaaattggaatacaactataactcacacaatgtatacatcatggcagacaaacaaaagaatggaatcaaagttaacttcaaaattagacacaacattgaagatggaagcgttcaactagcagaccattatcaacaaaatactccgattggcgatggccctgtccttttaccagacaaccattacctgtccacacaatctgccctttcgaaagatcccaacgaaaagagagaccacatggtccttcttgagtttgtaaccgctgctgggattacacatggcatggatgaactatacaaaaggcctgcagcaaacgacgaaaactacgctgcatcagtttaataataagataaaccagagcggcacggcaagcagagtatacgagattcggtagccaccgctgagcaataactagcataaccccttggggcctctaaacgggtcttgaggggttttttgcatatgcaacgg

SEQ ID NO: 84 - DNA, 1504 bp, Artificial Sequence
tcataagctttaatacgactcactataggctagttgtgttgtgtgtatgaagaaggccttgaataacggggtcttctttgtggttaaggaggaaaatatggcaaacctggacaagatgctgaataccacagtaacagaggtgcggcagttcctgcaggtggacagagtgtgcgtgttccagtttgaggaggattatagcggagtggtggtggtggaggccgtggacgataggtggatctccatcctgaagacccaggtgcgggatagatacttcatggagacaaggggcgaggagtattctcacggccgctaccaggccatcgccgacatctacaccgcaaacctgacagagtgctacagggatctgctgacacagtttcaggtgagagcaatcctggccgtgcccatcctgcagggcaagaagctgtggggcctgttggtggcacaccagctggcggcccctagacagtggcagacctgggagatcgactttctgaagcagcaggccgtggtggtgggcatcgccatccagcagagctaatttcctccttagtcacgaagaagacttctgactaaggagggaataatgtcgaagacgaacctggcggcagcgcaaaagatgcgtaaaggagaagaacttttcactggagttgtcccaattcttgttgaattagatggtgatgttaatgggcacaaattttctgtcagtggagagggtgaaggtgatgcaacatacggaaaacttacccttaaatttatttgcactactggaaaactacctgttccgtggccaacacttgtcactactttcggttatggtgttcaatgctttgcgagatacccagatcacatgaaacagcatgactttttcaagagtgccatgcccgaaggttacgtacaggaaagaactatatttttcaaagatgacgggaactacaagacacgtgctgaagtcaagtttgaaggtgatacccttgttaatagaatcgagttaaaaggtattgattttaaagaagatggaaacattcttggacacaaattggaatacaactataactcacacaatgtatacatcatggcagacaaacaaaagaatggaatcaaagttaacttcaaaattagacacaacattgaagatggaagcgttcaactagcagaccattatcaacaaaatactccgattggcgatggccctgtccttttaccagacaaccattacctgtccacacaatctgccctttcgaaagatcccaacgaaaagagagaccacatggtccttcttgagtttgtaaccgctgctgggattacacatggcatggatgaactatacaaaaggcctgcagcaaacgacgaaaactacgctgcatcagtttaataataagataaaccagagcggcacggcaagcagagtatacgagattcggtagccaccgctgagcaataactagcataaccccttggggcctctaaacgggtcttgaggggttttttgcatatgcaacgg

SEQ ID NO: 85 - DNA, 1504 bp, Artificial Sequence
tcataagctttaatacgactcactataggctagttgtgttgtgtgtatgaagaaggccttgaataacggggtcttcttcgtggttaaggaggaaaatatggcaaacctggacaagatgctgaataccacagtaacagaggtgcggcagttcctgcaggtggacagagtgtgcgtgttccagtttgaggaggattatagcggagtggtggtggtggaggccgtggacgataggtggatctccatcctgaagacccaggtgcgggatagatacttcatggagacaaggggcgaggagtattctcacggccgctaccaggccatcgccgacatctacaccgcaaacctgacagagtgctacagggatctgctgacacagtttcaggtgagagcaatcctggccgtgcccatcctgcagggcaagaagctgtggggcctgttggtggcacaccagctggcggcccctagacagtggcagacctgggagatcgactttctgaagcagcaggccgtggtggtgggcatcgccatccagcagagctaatttcctccttagtcacgaagaagacttctgactaaggagggaataatgtcgaagacgaacctggcggcagcgcaaaagatgcgtaaaggagaagaacttttcactggagttgtcccaattcttgttgaattagatggtgatgttaatgggcacaaattttctgtcagtggagagggtgaaggtgatgcaacatacggaaaacttacccttaaatttatttgcactactggaaaactacctgttccgtggccaacacttgtcactactttcggttatggtgttcaatgctttgcgagatacccagatcacatgaaacagcatgactttttcaagagtgccatgcccgaaggttacgtacaggaaagaactatatttttcaaagatgacgggaactacaagacacgtgctgaagtcaagtttgaaggtgatacccttgttaatagaatcgagttaaaaggtattgattttaaagaagatggaaacattcttggacacaaattggaatacaactataactcacacaatgtatacatcatggcagacaaacaaaagaatggaatcaaagttaacttcaaaattagacacaacattgaagatggaagcgttcaactagcagaccattatcaacaaaatactccgattggcgatggccctgtccttttaccagacaaccattacctgtccacacaatctgccctttcgaaagatcccaacgaaaagagagaccacatggtccttcttgagtttgtaaccgctgctgggattacacatggcatggatgaactatacaaaaggcctgcagcaaacgacgaaaactacgctgcatcagtttaataataagataaaccagagcggcacggcaagcagagtatacgagattcggtagccaccgctgagcaataactagcataaccccttggggcctctaaacgggtcttgaggggttttttgcatatgcaacgg

SEQ ID NO: 86 - DNA, 1504 bp, Artificial Sequence
tcataagctttaatacgactcactataggctagttgtgttgtgtgtatgaagagggccttgaataacggggtcttcttcgtggttaaggaggaaaatatggcaaacctggacaagatgctgaataccacagtaacagaggtgcggcagttcctgcaggtggacagagtgtgcgtgttccagtttgaggaggattatagcggagtggtggtggtggaggccgtggacgataggtggatctccatcctgaagacccaggtgcgggatagatacttcatggagacaaggggcgaggagtattctcacggccgctaccaggccatcgccgacatctacaccgcaaacctgacagagtgctacagggatctgctgacacagtttcaggtgagagcaatcctggccgtgcccatcctgcagggcaagaagctgtggggcctgttggtggcacaccagctggcggcccctagacagtggcagacctgggagatcgactttctgaagcagcaggccgtggtggtgggcatcgccatccagcagagctaatttcctccttagtcacgaagaagacttctgactaaggagggaataatgtcgaagacgaacctggcggcagcgcaaaagatgcgtaaaggagaagaacttttcactggagttgtcccaattcttgttgaattagatggtgatgttaatgggcacaaattttctgtcagtggagagggtgaaggtgatgcaacatacggaaaacttacccttaaatttatttgcactactggaaaactacctgttccgtggccaacacttgtcactactttcggttatggtgttcaatgctttgcgagatacccagatcacatgaaacagcatgactttttcaagagtgccatgcccgaaggttacgtacaggaaagaactatatttttcaaagatgacgggaactacaagacacgtgctgaagtcaagtttgaaggtgatacccttgttaatagaatcgagttaaaaggtattgattttaaagaagatggaaacattcttggacacaaattggaatacaactataactcacacaatgtatacatcatggcagacaaacaaaagaatggaatcaaagttaacttcaaaattagacacaacattgaagatggaagcgttcaactagcagaccattatcaacaaaatactccgattggcgatggccctgtccttttaccagacaaccattacctgtccacacaatctgccctttcgaaagatcccaacgaaaagagagaccacatggtccttcttgagtttgtaaccgctgctgggattacacatggcatggatgaactatacaaaaggcctgcagcaaacgacgaaaactacgctgcatcagtttaataataagataaaccagagcggcacggcaagcagagtatacgagattcggtagccaccgctgagcaataactagcataaccccttggggcctctaaacgggtcttgaggggttttttgcatatgcaacgg